European Patent Specification EP 3 607 053 B1, published August 26, 2026. Title: ANTIGEN-SPECIFIC T CELLS AND USES THEREOF. Applicant: Taipei Medical University. The sequence listing filed with the application follows.

SEQUENCE LISTING (143 sequences)

SEQ ID NO: 1 - DNA, 63 bp, Artificial Sequence
  Synthetic
atggagacagacacactcctgctatgggtactgctgctctgggttccaggttccactggtgac

SEQ ID NO: 2 - DNA, 645 bp, Artificial Sequence
  Synthetic
gacatcgtgatgacccagagccccagcagcctgagcgccagcgtgggcgacagagtgaccatcacctgcaaggccagccaggacgtgggcaccgccgtggactggtaccagcagaagcccggcaaggcccccaagctgctgatctactgggccagcaccagacacaccggcgtgcccgacagattcaccggcagcggcagcggcaccgacttcaccctgaccatcagcagcctgcagcccgaggacttcgccgactacttctgccagcagtacaacagctaccccctgaccttcggcggcggcaccaagctggagatcaagagaactgtggctgcaccatctgtcttcatcttcccgccatctgatgagcagttgaaatctggaactgcctctgttgtgtgcctgctgaataacttctatcccagagaggccaaagtacagtggaaggtggataacgccctccaatcgggtaactcccaggagagtgtcacagagcaggacagcaaggacagcacctacagcctcagcagcaccctgacgctgagcaaagcagactacgagaaacacaaactctacgcctgcgaagtcacccatcagggcctgagctcgcccgtcacaaagagcttcaacaggggagagtgctga

SEQ ID NO: 3 - DNA, 585 bp, Artificial Sequence
  Synthetic
gcccctctccctcccccccccctaacgttactggccgaagccgcttggaataaggccggtgtgcgtttgtctatatgttattttccaccatattgccgtcttttggcaatgtgagggcccggaaacctggccctgtcttcttgacgagcattcctaggggtctttcccctctcgccaaaggaatgcaaggtctgttgaatgtcgtgaaggaagcagttcctctggaagcttcttgaagacaaacaacgtctgtagcgaccctttgcaggcagcggaaccccccacctggcgacaggtgcctctgcggccaaaagccacgtgtataagatacacctgcaaaggcggcacaaccccagtgccacgttgtgagttggatagttgtggaaagagtcaaatggctctcctcaagcgtattcaacaaggggctgaaggatgcccagaaggtaccccattgtatgggatctgatctggggcctcggtgcacatgctttacatgtgtttagtcgaggttaaaaaaacgtctaggccccccgaaccacggggacgtggttttcctttgaaaaacacgatgataatatggccaca

SEQ ID NO: 4 - DNA, 660 bp, Artificial Sequence
  Synthetic
gaggtgcagctggtgcagagcggcgccgaggtgaagaagcccggcgccagcgtgaagatcagctgcaagaccagcggctacaccttcaccgagtacaccatccactgggtgaagcaggccagcggcaagggcctggagtggatcggcaacatcaaccccaacaacggcggcaccacctacaaccagaagttcgaggacagagccaccctgaccgtggacaagagcaccagcaccgcctacatggagctgagcagcctgagaagcgaggacaccgccgtgtactactgcgccgccggctggaacttcgactactggggccagggcaccaccgtgaccgtgagcagcgcctccaccaagggcccatcggtcttccccctggcaccctcctccaagagcacctctgggggcacagcggccctgggctgcctggtcaaggactacttccccgaaccggtgacggtgtcgtggaactcaggcgccctgaccagcggcgtgcacaccttcccggctgtcctacagtcctcaggactctactccctcagcagcgtggtgaccgtgccctccagcagcttgggcacccagacctacatctgcaacgtgaatcacaagcccagcaacaccaaggtggacaagagagttgagcccaaatcttgtgacaaa

SEQ ID NO: 5 - DNA, 774 bp, Artificial Sequence
  Synthetic
ggtggcggctcaggtggaggcgacatcaagctgcagcagagcggcgccgagctggccagacccggcgccagcgtgaagatgagctgcaagaccagcggctacaccttcaccagatacaccatgcactgggtgaagcagagacccggccagggcctggagtggatcggctacatcaaccccagcagaggctacaccaactacaaccagaagttcaaggacaaggccaccctgaccaccgacaagagcagcagcaccgcctacatgcagctgagcagcctgaccagcgaggacagcgccgtgtactactgcgccagatactacgacgaccactactgcctggactactggggccagggcaccaccctgaccgtgagcagcgtggagggcggcagcggcggcagcggcggcagcggcggcagcggcggcgtggacgacatccagctgacccagagccccgccatcatgagcgccagccccggcgagaaggtgaccatgacctgcagagccagcagcagcgtgagctacatgaactggtaccagcagaagagcggcaccagccccaagagatggatctacgacaccagcaaggtggccagcggcgtgccctacagattcagcggcagcggcagcggcaccagctacagcctgaccatcagcagcatggaggccgaggacgccgccacctactactgccagcagtggagcagcaaccccctgaccttcggcgctggcaccaagctggagctgaagagacaccaccaccaccaccactga

SEQ ID NO: 6 - DNA, 642 bp, Artificial Sequence
  Synthetic
gacatccagctgacccagagccccgccatcatgagcgccagccccggcgagaaggtgaccatgacctgcagagccagcagcagcgtgagctacatgaactggtaccagcagaagagcggcaccagccccaagagatggatctacgacaccagcaaggtggccagcggcgtgccctacagattcagcggcagcggcagcggcaccagctacagcctgaccatcagcagcatggaggccgaggacgccgccacctactactgccagcagtggagcagcaaccccctgaccttcggcgctggcaccaagctggagctgaagagaactgtggctgcaccatctgtcttcatcttcccgccatctgatgagcagttgaaatctggaactgcctctgttgtgtgcctgctgaataacttctatcccagagaggccaaagtacagtggaaggtggataacgccctccaatcgggtaactcccaggagagtgtcacagagcaggacagcaaggacagcacctacagcctcagcagcaccctgacgctgagcaaagcagactacgagaaacacaaactctacgcctgcgaagtcacccatcagggcctgagctcgcccgtcacaaagagcttcaacaggggagagtgctga

SEQ ID NO: 7 - DNA, 651 bp, Artificial Sequence
  Synthetic
gacatcaagctgcagcagagcggcgccgagctggccagacccggcgccagcgtgaagatgagctgcaagaccagcggctacaccttcaccagatacaccatgcactgggtgaagcagagacccggccagggcctggagtggatcggctacatcaaccccagcagaggctacaccaactacaaccagaagttcaaggacaaggccaccctgaccaccgacaagagcagcagcaccgcctacatgcagctgagcagcctgaccagcgaggacagcgccgtgtactactgcgccagatactacgacgaccactactgcctggactactggggccagggcaccaccctgaccgtgagcagcgcctccaccaaaggtccatcggtcttccccctggcgccctgctccaggagcacctccgagagcacagcggccctgggctgcctggtcaaggactacttccccgaaccggtgacggtgtcgtggaactcaggcgctctgaccagcggcgtgcacaccttcccagctgtcctacagtcctcaggactctactccctcagcagcgtggtgaccgtgccctccagcaacttcggcacccagacctacacctgcaacgtagatcacaagcccagtaacaccaaggtggacaagacagtt

SEQ ID NO: 8 - DNA, 759 bp, Artificial Sequence
  Synthetic
ggcggcggcagcggcggcggcgaggtgcagctggtgcagagcggcgccgaggtgaagaagcccggcgccagcgtgaagatcagctgcaagaccagcggctacaccttcaccgagtacaccatccactgggtgaagcaggccagcggcaagggcctggagtggatcggcaacatcaaccccaacaacggcggcaccacctacaaccagaagttcgaggacagagccaccctgaccgtggacaagagcaccagcaccgcctacatggagctgagcagcctgagaagcgaggacaccgccgtgtactactgcgccgccggctggaacttcgactactggggccagggcaccaccgtgaccgtgagcagcgccggtggaggcggttcaggcggaggtggctctggcggtggcggatcggacatcgtgatgacccagagccccagcagcctgagcgccagcgtgggcgacagagtgaccatcacctgcaaggccagccaggacgtgggcaccgccgtggactggtaccagcagaagcccggcaaggcccccaagctgctgatctactgggccagcaccagacacaccggcgtgcccgacagattcaccggcagcggcagcggcaccgacttcaccctgaccatcagcagcctgcagcccgaggacttcgccgactacttctgccagcagtacaacagctaccccctgaccttcggcggcggcaccaagctggagatcaagagacaccaccaccaccaccactga

SEQ ID NO: 9 - DNA, 717 bp, Artificial Sequence
  Synthetic
gacatcgtgatgacccagagccccagcagcctgagcgccagcgtgggcgacagagtgaccatcacctgcaaggccagccaggacgtgggcaccgccgtggactggtaccagcagaagcccggcaaggcccccaagctgctgatctactgggccagcaccagacacaccggcgtgcccgacagattcaccggcagcggcagcggcaccgacttcaccctgaccatcagcagcctgcagcccgaggacttcgccgactacttctgccagcagtacaacagctaccccctgaccttcggcggcggcaccaagctggagatcaagagaggtggaggcggttcaggcggaggtggctctggcggtggcggatcggaggtgcagctggtgcagagcggcgccgaggtgaagaagcccggcgccagcgtgaagatcagctgcaagaccagcggctacaccttcaccgagtacaccatccactgggtgaagcaggccagcggcaagggcctggagtggattggcaacatcaaccccaacaacggcggcaccacctacaaccagaagttcgaggacagagccaccctgaccgtggacaagagcaccagcaccgcctacatggagctgagcagcctgagaagcgaggacaccgccgtgtactactgcgccgctggctggaacttcgactactggggccagggcaccaccgtgaccgtgagcagcgcc

SEQ ID NO: 10 - DNA, 672 bp, Artificial Sequence
  Synthetic
gacatccagctgacccagagcccagcaatcatgtctgccagcccaggagagaaggtgaccatgacatgccgggccagcagcagcgtgagctacatgaactggtatcagcggaagagcggcacctcccctaagagatggatctacgacacatctaaggtggccagcggcgtgccatataggttctccggctctggcagcggcacctcctactctctgacaatcagctccatggaggccgaggatgccgccacctactattgccagcagtggtctagcaatcccctgacctttggcgccggcacaaagctggagctgaagaggaccgtggcagcacctagcgtgttcatctttcccccttccgacgagcagctgaagtccggcacagcctctgtggtgtgcctgctgaacaatttctatccacgcgaggccaaggtgcagtggaaggtggataacgccctgcagtctggcaatagccaggagtccgtgaccgagcaggactctaaggatagcacatactccctgtcctctaccctgacactgagcaaggccgattacgagaagcacaagctgtatgcatgcgaggtgacccaccagggcctgagctccccagtgacaaagtcttttaaccggggcgagtgtggcggcggctcccaccaccaccaccaccactga

SEQ ID NO: 11 - DNA, 1350 bp, Artificial Sequence
  Synthetic
gacatcaagctgcagcagagcggagcagagctggccaggcccggagcctctgtgaagatgagctgcaagacctccggctacaccttcacacggtatacaatgcactgggtgaagtacagacctggccagggcctggagtggatcggctatatcaacccatcccgcggctacaccaactataatcagaagtttaaggacaaggccaccctgaccacagataagagctcctctacagcctacatgcagctgagctccctgacctctgaggacagcgccgtgtactattgcgcccggtactatgacgatcactactgtctggattattggggccagggcaccacactgaccgtgtctagcgcctctacaaagggacctagcgtgttcccactggcaccctcctctaagtccacctctggaggaacagccgccctgggatgcctggtgaaggattacttcccagagcccgtgaccgtgtcctggaactctggcgccctgaccagcggagtgcacacatttcctgccgtgctgcagagctccggcctgtactccctgtctagcgtggtgacagtgccatcctctagcctgggcacccagacatatatctgcaacgtgaatcacaagccaagcaataccaaggtcgacaagaaggtggagcccaagtcctgtgataagacccacacatgccccccttgtcctgcaccagagctgctgggaggaccaagcgtgttcctgtttccacccaagcctaaggacaccctgatgatctctcggaccccagaggtgacatgcgtggtggtggacgtgagccacgaggatcccgaggtgaagtttaactggtacgtggatggcgtggaggtgcacaatgccaagaccaagcccagggaggagcagtacaattccacctatcgcgtggtgtctgtgctgacagtgctgcaccaggactggctgaacggcaaggagtataagtgcaaggtgtccaataaggccctgcccgcccctatcgagaagacaatctctaaggcaaagggacagcctcgggagccacaggtgtacaccctgcctccatccagagatgagctgaccaagaaccaggtgtctctgacatgtctggtgaagggcttctatccctctgacatcgccgtggagtgggagagcaatggccagcctgagaacaattacgataccacaccccctgtgctggacagcgatggctccttctttctgtatagcgacctgacagtggataagtccagatggcagcagggcaacgtgtttagctgttccgtgatgcacgaggccctgcacaatcactacacccagaagtctctgagcctgtcccccggcaagtaa

SEQ ID NO: 12 - DNA, 684 bp, Artificial Sequence
  Synthetic
aggatcgtgatgacccagtctcctagctccctgagcgcctccgtgggcgaccgcgtgaccatcacatgcaaggccagccaggatgtgggaaccgcagtggactggtaccaggataagccaggcaaggcccccaagctgctgatctattgggcctccaccaggcacacaggagtgccagacagattcaccggctctggcagcggcacagacttcaccctgacaatctctagcctgcagcccgaggacttcgccgattacttttgccagcagtacaacagctatcctctgaccttcggcggcggcacaaagctggagatcaagaggaccgtggcagcaccatccgtgttcatctttcccccttctgacgagcagctgaagtctggcacagccagcgtggtgtgctacctgaacaacttctaccccagggaggccaaggtgcagtggaaggtggataacgccctgcagtccggcaattctcaggagagcgtgaccgagcaggactccaaggattctacatacagcctgtggtccaccctgacactgtccaaggccgactacgagaagcacaagctgtatgcatgcgaggtgacccaccagggcctgtcctctcccgtgacaaagagcttcaataggggagagtgtggaggaggatcctacccttatgacgtgccagattatgcctaa

SEQ ID NO: 13 - DNA, 1338 bp, Artificial Sequence
  Synthetic
gaggtgcagctggtgcagtccggagcagaggtgaagaagcctggagcctctgtgaagatcagctgcaagacctccggctacaccttcacagagtatacaatccactgggtgaagaaggccagcggcaagggcctggagtggatcggcaacatcaatccaaacaatggcggcaccacatacaaccaggagtttgaggaccgggccaccctgacagtggataagtccacctctacagcctatatggagctgagctccctgagatccgaggacaccgccgtgtactattgcgccgccggctggaatttcgattactggggccagggcaccacagtgaccgtgtctagcgcctctacaaagggaccaagcgtgtttccactggcaccctcctctaagagcacctccggaggaacagccgccctgggctgtctggtgaaggactatttcccagagcccgtgaccgtgtcctggaactctggcgccctgacctccggagtggcaacaggaccagccgtgctgcagagctccggcctgtacagcctgtctagcgtggtgaccgtgccctcctctagcctgggcacccagacatatatctgcaacgtgaatcacaagccaagcaatacaaaggtcgacaagaaggtggagcccaagtcctgtgataagacccacacatgccccccttgtcctgcaccagagctgctgggaggaccaagcgtgttcctgtttccacccaagcctaaggacaccctgatgatctctaggacccccgaggtgacatgcgtggtggtggacgtgagccacgaggatcctgaggtgaagtttaactggtacgtggatggcgtggaggtgcacaatgccaagaccaagccccgggaggagcagtacaactccacctatagagtggtgtctgtgctgacagtgctgcaccaggactggctgaacggcaaggagtataagtgcaaggtgtccaataaggccctgcccgcccctatcgagaagaccatctctaaggccaagggccagcctagggagccacaggtgtacacactgcctccatcccgcaaggagctgaccaagaaccaggtgtctctgacatgtctggtgaagggcttctatccttctgatatcgccgtggagtgggagagcaatggccagccagagaacaattacaagaccacaccccctgtgctgaagagcgacggctccttctttctgtatagcaagctgaccgtggataagtccagatggcagcagggcaacgtgttttcttgtagcgtgatgcacgaggccctgcacaatcactacacacagaagtccctgtctctgagccctggcaagtaa

SEQ ID NO: 14 - DNA, 645 bp, Artificial Sequence
  Synthetic
gatattctgctgacccagagcccggttattctgagcgttagcccgggtgaacgtgttagctttagctgtcgtgcaagccagagcattggtaccaatattcattggtatcagcagcgtaccaatggtagcccgcgtctgctgattaaatatgcaagcgaaagcattagcggtattccgagccgttttagcggtagcggtagcggtaccgattttaccctgagcattaatagcgttgaaagcgaagatattgcagattattattgtcagcagaataataattggccgaccacctttggtgcaggtaccaaactggaactgaaacgtactgtggctgcaccatctgtcttcatcttcccgccatctgatgagcagttgaaatctggaactgcctctgttgtgtgcctgctgaataacttctatcccagagaggccaaagtacagtggaaggtggataacgccctccaatcgggtaactcccaggagagtgtcacagagcaggacagcaaggacagcacctacagcctcagcagcaccctgacgctgagcaaagcagactacgagaaacacaaactctacgcctgcgaagtcacccatcagggcctgagctcgcccgtcacaaagagcttcaacaggggagagtgctga

SEQ ID NO: 15 - DNA, 672 bp, Artificial Sequence
  Synthetic
caggttcagctgaaacagagcggtccgggtctggttcagccgagccagagcctgagcattacctgtaccgttagcggttttagcctgaccaattatggtgttcattgggttcgtcagagcccgggtaaaggtctggaatggctgggtgttatttggagcggtggtaataccgattataataccccgtttaccagccgtctgagcattaataaagataatagcaaaagccaggttttttttaaaatgaatagcctgcagagcaatgataccgcaatttattattgtgcacgtgcactgacctattatgattatgaatttgcatattggggtcagggtaccctggttaccgttagcgcagcctccaccaagggcccatcggtcttccccctggcaccctcctccaagagcacctctgggggcacagcggccctgggctgcctggtcaaggactacttccccgaaccggtgacggtgtcgtggaactcaggcgccctgaccagcggcgtgcacaccttcccggctgtcctacagtcctcaggactctactccctcagcagcgtggtgaccgtgccctccagcagcttgggcacccagacctacatctgcaacgtgaatcacaagcccagcaacaccaaggtggacaagagagttgagcccaaatcttgtgacaaa

SEQ ID NO: 16 - DNA, 768 bp, Artificial Sequence
  Synthetic
ggcggcggcagcggcggcggccaggttcagctgaaacagagcggtccgggtctggttcagccgagccagagcctgagcattacctgtaccgttagcggttttagcctgaccaattatggtgttcattgggttcgtcagagcccgggtaaaggtctggaatggctgggtgttatttggagcggtggtaataccgattataataccccgtttaccagccgtctgagcattaataaagataatagcaaaagccaggttttttttaaaatgaatagcctgcagagcaatgataccgcaatttattattgtgcacgtgcactgacctattatgattatgaatttgcatattggggtcagggtaccctggttaccgttagcgcaggcggcggcggcagcggcggcggcggcagcggcggcggcggcagcgatattctgctgacccagagcccggttattctgagcgttagcccgggtgaacgtgttagctttagctgtcgtgcaagccagagcattggtaccaatattcattggtatcagcagcgtaccaatggtagcccgcgtctgctgattaaatatgcaagcgaaagcattagcggtattccgagccgttttagcggtagcggtagcggtaccgattttaccctgagcattaatagcgttgaaagcgaagatattgcagattattattgtcagcagaataataattggccgaccacctttggtgcaggtaccaaactggaactgaaacgtcaccaccaccaccaccactga

SEQ ID NO: 17 - DNA, 726 bp, Artificial Sequence
  Synthetic
gatattctgctgacccagagcccggttattctgagcgttagcccgggtgaacgtgttagctttagctgtcgtgcaagccagagcattggtaccaatattcattggtatcagcagcgtaccaatggtagcccgcgtctgctgattaaatatgcaagcgaaagcattagcggtattccgagccgttttagcggtagcggtagcggtaccgattttaccctgagcattaatagcgttgaaagcgaagatattgcagattattattgtcagcagaataataattggccgaccacctttggtgcaggtaccaaactggaactgaaacgtggtggaggcggttcaggcggaggtggctctggcggtggcggatcgcaggttcagctgaaacagagcggtccgggtctggttcagccgagccagagcctgagcattacctgtaccgttagcggttttagcctgaccaattatggtgttcattgggttcgtcagagcccgggtaaaggtctggaatggctgggtgttatttggagcggtggtaataccgattataataccccgtttaccagccgtctgagcattaataaagataatagcaaaagccaggttttttttaaaatgaatagcctgcagagcaatgataccgcaatttattattgtgcacgtgcactgacctattatgattatgaatttgcatattggggtcagggtaccctggttaccgttagcgca

SEQ ID NO: 18 - DNA, 765 bp, Artificial Sequence
  Synthetic
ggcggtggatcagacatcaagctgcagcagagcggcgccgagctggccagacccggcgccagcgtgaagatgagctgcaagaccagcggctacaccttcaccagatacaccatgcactgggtgaagcagagacccggccagggcctggagtggatcggctacatcaaccccagcagaggctacaccaactacaaccagaagttcaaggacaaggccaccctgaccaccgacaagagcagcagcaccgcctacatgcagctgagcagcctgaccagcgaggacagcgccgtgtactactgcgccagatactacgacgaccactactgcctggactactggggccagggcaccaccctgaccgtgagcagcgtggagggcggcagcggcggcagcggcggcagcggcggcagcggcggcgtggacgacatccagctgacccagagccccgccatcatgagcgccagccccggcgagaaggtgaccatgacctgcagagccagcagcagcgtgagctacatgaactggtaccagcagaagagcggcaccagccccaagagatggatctacgacaccagcaaggtggccagcggcgtgccctacagattcagcggcagcggcagcggcaccagctacagcctgaccatcagcagcatggaggccgaggacgccgccacctactactgccagcagtggagcagcaaccccctgaccttcggcgctggcaccaagctggagctgaagagacaccaccaccaccaccactga

SEQ ID NO: 19 - DNA, 684 bp, Artificial Sequence
  Synthetic
aggattctgctgacccagagcccggttattctgagcgttagcccgggtgaacgtgttagctttagctgtcgtgcaagccagagcattggtaccaatattcattggtatcaggatcgtaccaatggtagcccgcgtctgctgattaaatatgcaagcgaaagcattagcggtattccgagccgttttagcggtagcggtagcggtaccgattttaccctgagcattaatagcgttgaaagcgaagatattgcagattattattgtcagcagaataataattggccgaccacctttggtgcaggtaccaaactggaactgaaacgtaccgtggcagcaccatccgtgttcatctttcccccttctgacgagcagctgaagtctggcacagccagcgtggtgtgctacctgaacaacttctaccccagggaggccaaggtgcagtggaaggtggataacgccctgcagtccggcaattctcaggagagcgtgaccgagcaggactccaaggattctacatacagcctgtggtccaccctgacactgtccaaggccgactacgagaagcacaagctgtatgcatgcgaggtgacccaccagggcctgtcctctcccgtgacaaagagcttcaataggggagagtgtggaggaggatcctacccttatgacgtgccagattatgcctaa

SEQ ID NO: 20 - DNA, 1350 bp, Artificial Sequence
  Synthetic
caggttcagctgaaacagagcggtccgggtctggttcagccgagccagagcctgagcattacctgtaccgttagcggttttagcctgaccaattatggtgttcattgggttcgtaagagcccgggtaaaggtctggaatggctgggtgttatttggagcggtggtaataccgattataataccgagtttaccagccgtctgagcattaataaagataatagcaaaagccaggttttttttaaaatgaatagcctgcagagcaatgataccgcaatttattattgtgcacgtgcactgacctattatgattatgaatttgcatattggggtcagggtaccctggttaccgttagcgcagcctctacaaagggaccaagcgtgtttccactggcaccctcctctaagagcacctccggaggaacagccgccctgggctgtctggtgaaggactatttcccagagcccgtgaccgtgtcctggaactctggcgccctgacctccggagtggcaacaggaccagccgtgctgcagagctccggcctgtacagcctgtctagcgtggtgaccgtgccctcctctagcctgggcacccagacatatatctgcaacgtgaatcacaagccaagcaatacaaaggtcgacaagaaggtggagcccaagtcctgtgataagacccacacatgccccccttgtcctgcaccagagctgctgggaggaccaagcgtgttcctgtttccacccaagcctaaggacaccctgatgatctctaggacccccgaggtgacatgcgtggtggtggacgtgagccacgaggatcctgaggtgaagtttaactggtacgtggatggcgtggaggtgcacaatgccaagaccaagccccgggaggagcagtacaactccacctatagagtggtgtctgtgctgacagtgctgcaccaggactggctgaacggcaaggagtataagtgcaaggtgtccaataaggccctgcccgcccctatcgagaagaccatctctaaggccaagggccagcctagggagccacaggtgtacacactgcctccatcccgcaaggagctgaccaagaaccaggtgtctctgacatgtctggtgaagggcttctatccttctgatatcgccgtggagtgggagagcaatggccagccagagaacaattacaagaccacaccccctgtgctgaagagcgacggctccttctttctgtatagcaagctgaccgtggataagtccagatggcagcagggcaacgtgttttcttgtagcgtgatgcacgaggccctgcacaatcactacacacagaagtccctgtctctgagccctggcaagtaa

SEQ ID NO: 21 - DNA, 645 bp, Artificial Sequence
  Synthetic
gatatccagatgacccagagccctagctccctgagcgcctccgtgggcgacagggtgaccatcacatgtagggcatcccaggacgtgagcaccgcagtggcctggtatcagcagaagcccggcaaggcccctaagctgctgatctactctgccagcttcctgtatagcggcgtgccttccagattttccggatctggaagcggaaccgacttcaccctgacaatctctagcctgcagccagaggattttgccacatactattgccagcagtacctgtatcacccagcaaccttcggacagggcacaaaagtggaaatcaagcggactgtggctgcaccatctgtcttcatcttcccgccatctgatgagcagttgaaatctggaactgcctctgttgtgtgcctgctgaataacttctatcccagagaggccaaagtacagtggaaggtggataacgccctccaatcgggtaactcccaggagagtgtcacagagcaggacagcaaggacagcacctacagcctcagcagcaccctgacgctgagcaaagcagactacgagaaacacaaactctacgcctgcgaagtcacccatcagggcctgagctcgcccgtcacaaagagcttcaacaggggagagtgctga

SEQ ID NO: 22 - DNA, 669 bp, Artificial Sequence
  Synthetic
gaggtgcagctggtggaaagcgggggaggactggtgcagcctggggggtcactgagactgagttgcgccgcctccggcttcaccttttccgactcttggatccactgggtgaggcaggcaccaggcaagggcctggagtgggtggcctggatctctccctacggcggcagcacctactatgccgactccgtgaagggccggtttacaatctctgccgataccagcaagaacacagcctatctgcagatgaattctctgagagccgaggacaccgccgtgtactattgcgcacggagacactggccaggaggattcgattactggggacagggcaccctggtgacagtgtccgccgcctccaccaagggcccatcggtcttccccctggcaccctcctccaagagcacctctgggggcacagcggccctgggctgcctggtcaaggactacttccccgaaccggtgacggtgtcgtggaactcaggcgccctgaccagcggcgtgcacaccttcccggctgtcctacagtcctcaggactctactccctcagcagcgtggtgaccgtgccctccagcagcttgggcacccagacctacatctgcaacgtgaatcacaagcccagcaacaccaaggtggacaagagagttgagcccaaatcttgtgacaaa

SEQ ID NO: 23 - DNA, 774 bp, Artificial Sequence
  Synthetic
gggggcgggagcgggggcggcgaggtgcagctggtggaaagcgggggaggactggtgcagcctggggggtcactgagactgagttgcgccgcctccggcttcaccttttccgactcttggatccactgggtgaggcaggcaccaggcaagggcctggagtgggtggcctggatctctccctacggcggcagcacctactatgccgactccgtgaagggccggtttacaatctctgccgataccagcaagaacacagcctatctgcagatgaattctctgagagccgaggacaccgccgtgtactattgcgcacggagacactggccaggaggattcgattactggggacagggcaccctggtgacagtgtccgccgtggagggaggatccggaggatctggaggaagcggcggctccggcggcgtggacgatatccagatgacccagagccctagctccctgagcgcctccgtgggcgacagggtgaccatcacatgtagggcatcccaggacgtgagcaccgcagtggcctggtatcagcagaagcccggcaaggcccctaagctgctgatctactctgccagcttcctgtatagcggcgtgccttccagattttccggatctggaagcggaaccgacttcaccctgacaatctctagcctgcagccagaggattttgccacatactattgccagcagtacctgtatcacccagcaaccttcggacagggcacaaaagtggaaatcaagcggcatcatcatcatcaccattaa

SEQ ID NO: 24 - DNA, 723 bp, Artificial Sequence
  Synthetic
gatatccagatgacccagagccctagctccctgagcgcctccgtgggcgacagggtgaccatcacatgtagggcatcccaggacgtgagcaccgcagtggcctggtatcagcagaagcccggcaaggcccctaagctgctgatctactctgccagcttcctgtatagcggcgtgccttccagattttccggatctggaagcggaaccgacttcaccctgacaatctctagcctgcagccagaggattttgccacatactattgccagcagtacctgtatcacccagcaaccttcggacagggcacaaaagtggaaatcaagcggggtggaggcggttcaggcggaggtggctctggcggtggcggatcggaggtgcagctggtggaaagcgggggaggactggtgcagcctggggggtcactgagactgagttgcgccgcctccggcttcaccttttccgactcttggatccactgggtgaggcaggcaccaggcaagggcctggagtgggtggcctggatctctccctacggcggcagcacctactatgccgactccgtgaagggccggtttacaatctctgccgataccagcaagaacacagcctatctgcagatgaattctctgagagccgaggacaccgccgtgtactattgcgcacggagacactggccaggaggattcgattactggggacagggcaccctggtgacagtgtccgcc

SEQ ID NO: 25 - DNA, 684 bp, Artificial Sequence
  Synthetic
aggatccagatgacccagagccctagctccctgagcgcctccgtgggcgacagggtgaccatcacatgtagggcatcccaggacgtgagcaccgcagtggcctggtatcaggataagcccggcaaggcccctaagctgctgatctactctgccagcttcctgtatagcggcgtgccttccagattttccggatctggaagcggaaccgacttcaccctgacaatctctagcctgcagccagaggattttgccacatactattgccagcagtacctgtatcacccagcaaccttcggacagggcacaaaagtggaaatcaagcggaccgtggcagcaccatccgtgttcatctttcccccttctgacgagcagctgaagtctggcacagccagcgtggtgtgctacctgaacaacttctaccccagggaggccaaggtgcagtggaaggtggataacgccctgcagtccggcaattctcaggagagcgtgaccgagcaggactccaaggattctacatacagcctgtggtccaccctgacactgtccaaggccgactacgagaagcacaagctgtatgcatgcgaggtgacccaccagggcctgtcctctcccgtgacaaagagcttcaataggggagagtgtggaggaggatcctacccttatgacgtgccagattatgcctaa

SEQ ID NO: 26 - DNA, 1347 bp, Artificial Sequence
  Synthetic
gaggtgcagctggtggaaagcgggggaggactggtgcagcctggggggtcactgagactgagttgcgccgcctccggcttcaccttttccgactcttggatccactgggtgaggaaggcaccaggcaagggcctggagtgggtggcctggatctctccctacggcggcagcacctactatgccgactccgtgaagggcgagtttacaatctctgccgataccagcaagaacacagcctatctgcagatgaattctctgagagccgaggacaccgccgtgtactattgcgcacggagacactggccaggaggattcgattactggggacagggcaccctggtgacagtgtccgccgcctctacaaagggaccaagcgtgtttccactggcaccctcctctaagagcacctccggaggaacagccgccctgggctgtctggtgaaggactatttcccagagcccgtgaccgtgtcctggaactctggcgccctgacctccggagtggcaacaggaccagccgtgctgcagagctccggcctgtacagcctgtctagcgtggtgaccgtgccctcctctagcctgggcacccagacatatatctgcaacgtgaatcacaagccaagcaatacaaaggtcgacaagaaggtggagcccaagtcctgtgataagacccacacatgccccccttgtcctgcaccagagctgctgggaggaccaagcgtgttcctgtttccacccaagcctaaggacaccctgatgatctctaggacccccgaggtgacatgcgtggtggtggacgtgagccacgaggatcctgaggtgaagtttaactggtacgtggatggcgtggaggtgcacaatgccaagaccaagccccgggaggagcagtacaactccacctatagagtggtgtctgtgctgacagtgctgcaccaggactggctgaacggcaaggagtataagtgcaaggtgtccaataaggccctgcccgcccctatcgagaagaccatctctaaggccaagggccagcctagggagccacaggtgtacacactgcctccatcccgcaaggagctgaccaagaaccaggtgtctctgacatgtctggtgaagggcttctatccttctgatatcgccgtggagtgggagagcaatggccagccagagaacaattacaagaccacaccccctgtgctgaagagcgacggctccttctttctgtatagcaagctgaccgtggataagtccagatggcagcagggcaacgtgttttcttgtagcgtgatgcacgaggccctgcacaatcactacacacagaagtccctgtctctgagccctggcaagtaa

SEQ ID NO: 27 - DNA, 645 bp, Artificial Sequence
  Synthetic
gacatccagatgacccagagccccagcagcctgagcgccagcgtgggcgacagagtgaccatcacctgcagagccagccaggacgtgaacaccgccgtggcctggtaccagcagaagcccggcaaggcccccaagctgctgatctacagcgccagcttcctgtacagcggcgtgcccagcagattcagcggcagcagaagcggcaccgacttcaccctgaccatcagcagcctgcagcccgaggacttcgccacctactactgccagcagcactacaccaccccccccaccttcggccagggcaccaaggtggagatcaagagaactgtggctgcaccatctgtcttcatcttcccgccatctgatgagcagttgaaatctggaactgcctctgttgtgtgcctgctgaataacttctatcccagagaggccaaagtacagtggaaggtggataacgccctccaatcgggtaactcccaggagagtgtcacagagcaggacagcaaggacagcacctacagcctcagcagcaccctgacgctgagcaaagcagactacgagaaacacaaactctacgcctgcgaagtcacccatcagggcctgagctcgcccgtcacaaagagcttcaacaggggagagtgctga

SEQ ID NO: 28 - DNA, 675 bp, Artificial Sequence
  Synthetic
gaggtgcagctggtggagagcggcggcggcctggtgcagcccggcggcagcctgagactgagctgcgccgccagcggcttcaacatcaaggacacctacatccactgggtgagacaggcccccggcaagggcctggagtgggtggccagaatctaccccaccaacggctacaccagatacgccgacagcgtgaagggcagattcaccatcagcgccgacaccagcaagaacaccgcctacctgcagatgaacagcctgagagccgaggacaccgccgtgtactactgcagcagatggggcggcgacggcttctacgccatggactactggggccagggcaccctggtgaccgtgagcagcgcctccaccaagggcccatcggtcttccccctggcaccctcctccaagagcacctctgggggcacagcggccctgggctgcctggtcaaggactacttccccgaaccggtgacggtgtcgtggaactcaggcgccctgaccagcggcgtgcacaccttcccggctgtcctacagtcctcaggactctactccctcagcagcgtggtgaccgtgccctccagcagcttgggcacccagacctacatctgcaacgtgaatcacaagcccagcaacaccaaggtggacaagagagttgagcccaaatcttgtgacaaa

SEQ ID NO: 29 - DNA, 759 bp, Artificial Sequence; identical to SEQ ID NO: 8
  Synthetic

SEQ ID NO: 30 - DNA, 729 bp, Artificial Sequence
  Synthetic
gacatccagatgacccagagccccagcagcctgagcgccagcgtgggcgacagagtgaccatcacctgcagagccagccaggacgtgaacaccgccgtggcctggtaccagcagaagcccggcaaggcccccaagctgctgatctacagcgccagcttcctgtacagcggcgtgcccagcagattcagcggcagcagaagcggcaccgacttcaccctgaccatcagcagcctgcagcccgaggacttcgccacctactactgccagcagcactacaccaccccccccaccttcggccagggcaccaaggtggagatcaagagaggtggaggcggttcaggcggaggtggctctggcggtggcggatcggaggtgcagctggtggagagcggcggcggcctggtgcagcccggcggcagcctgagactgagctgcgccgccagcggcttcaacatcaaggacacctacatccactgggtgagacaggcccccggcaagggcctggagtgggtggccagaatctaccccaccaacggctacaccagatacgccgacagcgtgaagggcagattcaccatcagcgccgacaccagcaagaacaccgcctacctgcagatgaacagcctgagagccgaggacaccgccgtgtactactgcagcagatggggcggcgacggcttctacgccatggactactggggccagggcaccctggtgaccgtgagcagc

SEQ ID NO: 31 - DNA, 684 bp, Artificial Sequence
  Synthetic
aggatccagatgacccagagccccagcagcctgagcgccagcgtgggcgacagagtgaccatcacctgcagagccagccaggacgtgaacaccgccgtggcctggtaccaggataagcccggcaaggcccccaagctgctgatctacagcgccagcttcctgtacagcggcgtgcccagcagattcagcggcagcagaagcggcaccgacttcaccctgaccatcagcagcctgcagcccgaggacttcgccacctactactgccagcagcactacaccaccccccccaccttcggccagggcaccaaggtggagatcaagagaaccgtggcagcaccatccgtgttcatctttcccccttctgacgagcagctgaagtctggcacagccagcgtggtgtgctacctgaacaacttctaccccagggaggccaaggtgcagtggaaggtggataacgccctgcagtccggcaattctcaggagagcgtgaccgagcaggactccaaggattctacatacagcctgtggtccaccctgacactgtccaaggccgactacgagaagcacaagctgtatgcatgcgaggtgacccaccagggcctgtcctctcccgtgacaaagagcttcaataggggagagtgtggaggaggatcctacccttatgacgtgccagattatgcctaa

SEQ ID NO: 32 - DNA, 1353 bp, Artificial Sequence
  Synthetic
gaggtgcagctggtggagagcggcggcggcctggtgcagcccggcggcagcctgagactgagctgcgccgccagcggcttcaacatcaaggacacctacatccactgggtgagaaaggcccccggcaagggcctggagtgggtggccagaatctaccccaccaacggctacaccagatacgccgacagcgtgaagggcaggttcaccatcagcgccgacaccagcaagaacaccgcctacctgcagatgaacagcctgagagccgaggacaccgccgtgtactactgcagcagatggggcggcgacggcttctacgccatggactactggggccagggcaccctggtgaccgtgagcagcgcctctacaaagggaccaagcgtgtttccactggcaccctcctctaagagcacctccggaggaacagccgccctgggctgtctggtgaaggactatttcccagagcccgtgaccgtgtcctggaactctggcgccctgacctccggagtggcaacaggaccagccgtgctgcagagctccggcctgtacagcctgtctagcgtggtgaccgtgccctcctctagcctgggcacccagacatatatctgcaacgtgaatcacaagccaagcaatacaaaggtcgacaagaaggtggagcccaagtcctgtgataagacccacacatgccccccttgtcctgcaccagagctgctgggaggaccaagcgtgttcctgtttccacccaagcctaaggacaccctgatgatctctaggacccccgaggtgacatgcgtggtggtggacgtgagccacgaggatcctgaggtgaagtttaactggtacgtggatggcgtggaggtgcacaatgccaagaccaagccccgggaggagcagtacaactccacctatagagtggtgtctgtgctgacagtgctgcaccaggactggctgaacggcaaggagtataagtgcaaggtgtccaataaggccctgcccgcccctatcgagaagaccatctctaaggccaagggccagcctagggagccacaggtgtacacactgcctccatcccgcaaggagctgaccaagaaccaggtgtctctgacatgtctggtgaagggcttctatccttctgatatcgccgtggagtgggagagcaatggccagccagagaacaattacaagaccacaccccctgtgctgaagagcgacggctccttctttctgtatagcaagctgaccgtggataagtccagatggcagcagggcaacgtgttttcttgtagcgtgatgcacgaggccctgcacaatcactacacacagaagtccctgtctctgagccctggcaagtaa

SEQ ID NO: 33 - DNA, 660 bp, Artificial Sequence
  Synthetic
gacattgtgatgacccagtcccctgacagcctggctgtgagcctgggagagagggccaccatcaactgcaagagcagccagagcctgctgtacagcagaaaccagaaaaactacctggcctggtaccagcagaaacccggccagcctcccaagctgctgatcttctgggccagcaccagagagagcggcgtgcctgacagattcagcggctccggcttcggcaccgacttcaccctgaccatcagcagcctccaggccgaggatgtcgccgtgtattactgccagcagtacttctcctatcccctcaccttcggccaaggcaccaaggtggagatcaagactgtggctgcaccatctgtcttcatcttcccgccatctgatgagcagttgaaatctggaactgcctctgttgtgtgcctgctgaataacttctatcccagagaggccaaagtacagtggaaggtggataacgccctccaatcgggtaactcccaggagagtgtcacagagcaggacagcaaggacagcacctacagcctcagcagcaccctgacgctgagcaaagcagactacgagaaacacaaactctacgcctgcgaagtcacccatcagggcctgagctcgcccgtcacaaagagcttcaacaggggagagtgctga

SEQ ID NO: 34 - DNA, 687 bp, Artificial Sequence
  Synthetic
caagtgcagctggtgcagtccggcgctgaggtgaagaagcccggagcctccgtgaaggtgtcctgcaagacctccaggtacaccttcacagagtacaccatccactgggtgagacaggctcccggccagaggctggagtggattggcggcattaaccccaacaacggcatccccaactacaaccagaagttcaagggcagggtgaccatcacagttgatacatccgccagcacagcctatatggaactgagctccctgaggagcgaggacacagccgtgtactactgcgccaggaggaggattgcctacggctatgatgagggccatgccatggactactggggacagggcaccctggtgacagtctccagcgcctccaccaagggcccatcggtcttccccctggcaccctcctccaagagcacctctgggggcacagcggccctgggctgcctggtcaaggactacttccccgaaccggtgacggtgtcgtggaactcaggcgccctgaccagcggcgtgcacaccttcccggctgtcctacagtcctcaggactctactccctcagcagcgtggtgaccgtgccctccagcagcttgggcacccagacctacatctgcaacgtgaatcacaagcccagcaacaccaaggtggacaagagagttgagcccaaatcttgtgacaaa

SEQ ID NO: 35 - DNA, 807 bp, Artificial Sequence
  Synthetic
ggcggcggcagcggcggcggccaagtgcagctggtgcagtccggcgctgaggtgaagaagcccggagcctccgtgaaggtgtcctgcaagacctccaggtacaccttcacagagtacaccatccactgggtgagacaggctcccggccagaggctggagtggattggcggcattaaccccaacaacggcatccccaactacaaccagaagttcaagggcagggtgaccatcacagttgatacatccgccagcacagcctatatggaactgagctccctgaggagcgaggacacagccgtgtactactgcgccaggaggaggattgcctacggctatgatgagggccatgccatggactactggggacagggcaccctggtgacagtctccagcggcagcaccagcggatccggaaagcctggcagcggagagggaagcaccaagggcgacattgtgatgacccagtcccctgacagcctggctgtgagcctgggagagagggccaccatcaactgcaagagcagccagagcctgctgtacagcagaaaccagaaaaactacctggcctggtaccagcagaaacccggccagcctcccaagctgctgatcttctgggccagcaccagagagagcggcgtgcctgacagattcagcggctccggcttcggcaccgacttcaccctgaccatcagcagcctccaggccgaggatgtcgccgtgtattactgccagcagtacttctcctatcccctcaccttcggccaaggcaccaaggtggagatcaagcaccaccaccaccaccactga

SEQ ID NO: 36 - DNA, 756 bp, Artificial Sequence
  Synthetic
gacattgtgatgacccagtcccctgacagcctggctgtgagcctgggagagagggccaccatcaactgcaagagcagccagagcctgctgtacagcagaaaccagaaaaactacctggcctggtaccagcagaaacccggccagcctcccaagctgctgatcttctgggccagcaccagagagagcggcgtgcctgacagattcagcggctccggcttcggcaccgacttcaccctgaccatcagcagcctccaggccgaggatgtcgccgtgtattactgccagcagtacttctcctatcccctcaccttcggccaaggcaccaaggtggagatcaagggtggaggcggttcaggcggaggtggctctggcggtggcggatcgcaagtgcagctggtgcagtccggcgctgaggtgaagaagcccggagcctccgtgaaggtgtcctgcaagacctccaggtacaccttcacagagtacaccatccactgggtgagacaggctcccggccagaggctggagtggattggcggcattaaccccaacaacggcatccccaactacaaccagaagttcaagggcagggtgaccatcacagttgatacatccgccagcacagcctatatggaactgagctccctgaggagcgaggacacagccgtgtactactgcgccaggaggaggattgcctacggctatgatgagggccatgccatggactactggggacagggcaccctggtgacagtctccagc

SEQ ID NO: 37 - DNA, 699 bp, Artificial Sequence
  Synthetic
aggattgtgatgacccagtcccctgacagcctggctgtgagcctgggagagagggccaccatcaactgcaagagcagccagagcctgctgtacagcagaaaccagaaaaactacctggcctggtaccaggataaacccggccagcctcccaagctgctgatcttctgggccagcaccagagagagcggcgtgcctgacagattcagcggctccggcttcggcaccgacttcaccctgaccatcagcagcctccaggccgaggatgtcgccgtgtattactgccagcagtacttctcctatcccctcaccttcggccaaggcaccaaggtggagatcaagaccgtggcagcaccatccgtgttcatctttcccccttctgacgagcagctgaagtctggcacagccagcgtggtgtgctacctgaacaacttctaccccagggaggccaaggtgcagtggaaggtggataacgccctgcagtccggcaattctcaggagagcgtgaccgagcaggactccaaggattctacatacagcctgtggtccaccctgacactgtccaaggccgactacgagaagcacaagctgtatgcatgcgaggtgacccaccagggcctgtcctctcccgtgacaaagagcttcaataggggagagtgtggaggaggatcctacccttatgacgtgccagattatgcctaa

SEQ ID NO: 38 - DNA, 1365 bp, Artificial Sequence
  Synthetic
caagtgcagctggtgcagtccggcgctgaggtgaagaagcccggagcctccgtgaaggtgtcctgcaagacctccaggtacaccttcacagagtacaccatccactgggtgagaaaggctcccggccagaggctggagtggattggcggcattaaccccaacaacggcatccccaactacaaccagaggttcaagggcagggtgaccatcacagttgatacatccgccagcacagcctatatggaactgagctccctgaggagcgaggacacagccgtgtactactgcgccaggaggaggattgcctacggctatgatgagggccatgccatggactactggggacagggcaccctggtgacagtctccagcgcctctacaaagggaccaagcgtgtttccactggcaccctcctctaagagcacctccggaggaacagccgccctgggctgtctggtgaaggactatttcccagagcccgtgaccgtgtcctggaactctggcgccctgacctccggagtggcaacaggaccagccgtgctgcagagctccggcctgtacagcctgtctagcgtggtgaccgtgccctcctctagcctgggcacccagacatatatctgcaacgtgaatcacaagccaagcaatacaaaggtcgacaagaaggtggagcccaagtcctgtgataagacccacacatgccccccttgtcctgcaccagagctgctgggaggaccaagcgtgttcctgtttccacccaagcctaaggacaccctgatgatctctaggacccccgaggtgacatgcgtggtggtggacgtgagccacgaggatcctgaggtgaagtttaactggtacgtggatggcgtggaggtgcacaatgccaagaccaagccccgggaggagcagtacaactccacctatagagtggtgtctgtgctgacagtgctgcaccaggactggctgaacggcaaggagtataagtgcaaggtgtccaataaggccctgcccgcccctatcgagaagaccatctctaaggccaagggccagcctagggagccacaggtgtacacactgcctccatcccgcaaggagctgaccaagaaccaggtgtctctgacatgtctggtgaagggcttctatccttctgatatcgccgtggagtgggagagcaatggccagccagagaacaattacaagaccacaccccctgtgctgaagagcgacggctccttctttctgtatagcaagctgaccgtggataagtccagatggcagcagggcaacgtgttttcttgtagcgtgatgcacgaggccctgcacaatcactacacacagaagtccctgtctctgagccctggcaagtaa

SEQ ID NO: 39 - DNA, 657 bp, Artificial Sequence
  Synthetic
gatattcagatgacccagagcccttcaagcctgtccgccagcgtcggggatagagtgaccattacttgccggagcaccaagtccctgctgcactccaacggcatcacatacctgtattggtaccagcagaagcccggcaaggcccctaagctgctgatctatcagatgtccaatctggcctctggcgtgccaagcagattcagctcctctggcagcggcaccgactttaccctgacaatcagctccctgcagcccgaggatttcgccacatactattgcgcccagaacctggagatccctaggacctttggccagggcacaaaggtggagctgaagactgtggctgcaccatctgtcttcatcttcccgccatctgatgagcagttgaaatctggaactgcctctgttgtgtgcctgctgaataacttctatcccagagaggccaaagtacagtggaaggtggataacgccctccaatcgggtaactcccaggagagtgtcacagagcaggacagcaaggacagcacctacagcctcagcagcaccctgacgctgagcaaagcagactacgagaaacacaaactctacgcctgcgaagtcacccatcagggcctgagctcgcccgtcacaaagagcttcaacaggggagagtgctga

SEQ ID NO: 40 - DNA, 663 bp, Artificial Sequence
  Synthetic
gaggtgcagctggtgcagtccggacctggcctggtgcagccaggaggctccgtgaggatctcttgtgccgccagcggctataccttcacaaactacggcatgaattgggtgaagcaggcacctggcaagggcctggagtggatgggctggatcaacacctatacaggcgagtccacctacgccgactcttttaagggcagattcaccttttctctggatacatccgcctctgccgcctacctgcagatcaatagcctgcgggccgaggacacagccgtgtactattgtgccagattcgccatcaaaggggactactggggacagggcacactgctgaccgtctcaagcgcctccaccaagggcccatcggtcttccccctggcaccctcctccaagagcacctctgggggcacagcggccctgggctgcctggtcaaggactacttccccgaaccggtgacggtgtcgtggaactcaggcgccctgaccagcggcgtgcacaccttcccggctgtcctacagtcctcaggactctactccctcagcagcgtggtgaccgtgccctccagcagcttgggcacccagacctacatctgcaacgtgaatcacaagcccagcaacaccaaggtggacaagagagttgagcccaaatcttgtgacaaa

SEQ ID NO: 41 - DNA, 771 bp, Artificial Sequence
  Synthetic
ggcggcggcagcggcggcggcgaggtgcagctggtgcagtccggacctggcctggtgcagccaggaggctccgtgaggatctcttgtgccgccagcggctataccttcacaaactacggcatgaattgggtgaagcaggcacctggcaagggcctggagtggatgggctggatcaacacctatacaggcgagtccacctacgccgactcttttaagggcagattcaccttttctctggatacatccgcctctgccgcctacctgcagatcaatagcctgcgggccgaggacacagccgtgtactattgtgccagattcgccatcaaaggggactactggggacagggcacactgctgaccgtctcaagcggtggaggcggttcaggcggaggtggctctggcggtggcggatcggatattcagatgacccagagcccttcaagcctgtccgccagcgtcggggatagagtgaccattacttgccggagcaccaagtccctgctgcactccaacggcatcacatacctgtattggtaccagcagaagcccggcaaggcccctaagctgctgatctatcagatgtccaatctggcctctggcgtgccaagcagattcagctcctctggcagcggcaccgactttaccctgacaatcagctccctgcagcccgaggatttcgccacatactattgcgcccagaacctggagatccctaggacctttggccagggcacaaaggtggagctgaagcaccaccaccaccaccactga

SEQ ID NO: 42 - DNA, 762 bp, Artificial Sequence
  Synthetic
gatattcagatgacccagagcccttcaagcctgtccgccagcgtcggggatagagtgaccattacttgccggagcaccaagtccctgctgcactccaacggcatcacatacctgtattggtaccagcagaagcccggcaaggcccctaagctgctgatctatcagatgtccaatctggcctctggcgtgccaagcagattcagctcctctggcagcggcaccgactttaccctgacaatcagctccctgcagcccgaggatttcgccacatactattgcgcccagaacctggagatccctaggacctttggccagggcacaaaggtggagctgaagcgcgccaccccctctcacaacagccaccaggtgccaagcgccggaggaccaaccgccaattccggcacatctggaagcgaggtgcagctggtgcagtccggacctggcctggtgcagccaggaggctccgtgaggatctcttgtgccgccagcggctataccttcacaaactacggcatgaattgggtgaagcaggcacctggcaagggcctggagtggatgggctggatcaacacctatacaggcgagtccacctacgccgactcttttaagggcagattcaccttttctctggatacatccgcctctgccgcctacctgcagatcaatagcctgcgggccgaggacacagccgtgtactattgtgccagattcgccatcaaaggggactactggggacagggcacactgctgaccgtctcaagc

SEQ ID NO: 43 - DNA, 696 bp, Artificial Sequence
  Synthetic
aggattcagatgacccagagcccttcaagcctgtccgccagcgtcggggatagagtgaccattacttgccggagcaccaagtccctgctgcactccaacggcatcacatacctgtattggtaccaggataagcccggcaaggcccctaagctgctgatctatcagatgtccaatctggcctctggcgtgccaagcagattcagctcctctggcagcggcaccgactttaccctgacaatcagctccctgcagcccgaggatttcgccacatactattgcgcccagaacctggagatccctaggacctttggccagggcacaaaggtggagctgaagaccgtggcagcaccatccgtgttcatctttcccccttctgacgagcagctgaagtctggcacagccagcgtggtgtgctacctgaacaacttctaccccagggaggccaaggtgcagtggaaggtggataacgccctgcagtccggcaattctcaggagagcgtgaccgagcaggactccaaggattctacatacagcctgtggtccaccctgacactgtccaaggccgactacgagaagcacaagctgtatgcatgcgaggtgacccaccagggcctgtcctctcccgtgacaaagagcttcaataggggagagtgtggaggaggatcctacccttatgacgtgccagattatgcctaa

SEQ ID NO: 44 - DNA, 1341 bp, Artificial Sequence
  Synthetic
gaggtgcagctggtgcagtccggacctggcctggtgcagccaggaggctccgtgaggatctcttgtgccgccagcggctataccttcacaaactacggcatgaattgggtgaagaaggcacctggcaagggcctggagtggatgggctggatcaacacctatacaggcgagtccacctacgccgactcttttaagggcgagttcaccttttctctggatacatccgcctctgccgcctacctgcagatcaatagcctgcgggccgaggacacagccgtgtactattgtgccagattcgccatcaaaggggactactggggacagggcacactgctgaccgtctcaagcgcctctacaaagggaccaagcgtgtttccactggcaccctcctctaagagcacctccggaggaacagccgccctgggctgtctggtgaaggactatttcccagagcccgtgaccgtgtcctggaactctggcgccctgacctccggagtggcaacaggaccagccgtgctgcagagctccggcctgtacagcctgtctagcgtggtgaccgtgccctcctctagcctgggcacccagacatatatctgcaacgtgaatcacaagccaagcaatacaaaggtcgacaagaaggtggagcccaagtcctgtgataagacccacacatgccccccttgtcctgcaccagagctgctgggaggaccaagcgtgttcctgtttccacccaagcctaaggacaccctgatgatctctaggacccccgaggtgacatgcgtggtggtggacgtgagccacgaggatcctgaggtgaagtttaactggtacgtggatggcgtggaggtgcacaatgccaagaccaagccccgggaggagcagtacaactccacctatagagtggtgtctgtgctgacagtgctgcaccaggactggctgaacggcaaggagtataagtgcaaggtgtccaataaggccctgcccgcccctatcgagaagaccatctctaaggccaagggccagcctagggagccacaggtgtacacactgcctccatcccgcaaggagctgaccaagaaccaggtgtctctgacatgtctggtgaagggcttctatccttctgatatcgccgtggagtgggagagcaatggccagccagagaacaattacaagaccacaccccctgtgctgaagagcgacggctccttctttctgtatagcaagctgaccgtggataagtccagatggcagcagggcaacgtgttttcttgtagcgtgatgcacgaggccctgcacaatcactacacacagaagtccctgtctctgagccctggcaagtaa

SEQ ID NO: 45 - DNA, 642 bp, Artificial Sequence
  Synthetic
gagctgcagatgacccagtcccctagctctttaagcgcttccgtgggcgacagagtgaccatcacatgtcgtacctcccagagcatcagctcctatttaaactggtaccagcagaagcccggacagccccccaagctgctgatctactgggcttccactcgtgaaagcggcgtgcccgatcgtttttccggcagcggcagcggcaccgactttactttaaccatctcctctttacagcccgaggatagcgccacctactactgccagcagagctacgacatcccctacacattcggccaaggtaccaagctggaaatcaaaactgtggctgcaccatctgtcttcatcttcccgccatctgatgagcagttgaaatctggaactgcctctgttgtgtgcctgctgaataacttctatcccagagaggccaaagtacagtggaaggtggataacgccctccaatcgggtaactcccaggagagtgtcacagagcaggacagcaaggacagcacctacagcctcagcagcaccctgacgctgagcaaagcagactacgagaaacacaaactctacgcctgcgaagtcacccatcagggcctgagctcgcccgtcacaaagagcttcaacaggggagagtgctga

SEQ ID NO: 46 - DNA, 696 bp, Artificial Sequence
  Synthetic
gaagtgcagctgctggagagcggaggcggagtggtgcaacccggtcgttctttaaggctgagctgcgctgccagcggcttcaccttcagcagctatggcatgcactgggtgagacaagctcccggaaaaggtttagagtgggtggccgtgatctcctacgacggcagcaacaagtactacgccgacagcgtgaagggtcgtttcaccatctctcgtgacaactccaagaacactttatacctccagatgaactctttaagggccgaggacaccgccgtgtactactgtgccaaggacatgggctggggcagcggatggaggccctactactactacggcatggacgtgtggggccaaggtacaaccgtgaccgtgtccagcgcctccaccaagggcccatcggtcttccccctggcaccctcctccaagagcacctctgggggcacagcggccctgggctgcctggtcaaggactacttccccgaaccggtgacggtgtcgtggaactcaggcgccctgaccagcggcgtgcacaccttcccggctgtcctacagtcctcaggactctactccctcagcagcgtggtgaccgtgccctccagcagcttgggcacccagacctacatctgcaacgtgaatcacaagcccagcaacaccaaggtggacaagagagttgagcccaaatcttgtgacaaa

SEQ ID NO: 47 - DNA, 789 bp, Artificial Sequence
  Synthetic
ggcggcggcagcggcggcggcgaagtgcagctgctggagagcggaggcggagtggtgcaacccggtcgttctttaaggctgagctgcgctgccagcggcttcaccttcagcagctatggcatgcactgggtgagacaagctcccggaaaaggtttagagtgggtggccgtgatctcctacgacggcagcaacaagtactacgccgacagcgtgaagggtcgtttcaccatctctcgtgacaactccaagaacactttatacctccagatgaactctttaagggccgaggacaccgccgtgtactactgtgccaaggacatgggctggggcagcggatggaggccctactactactacggcatggacgtgtggggccaaggtacaaccgtgaccgtgtccagcggtggaggcggttcaggcggaggtggctctggcggtggcggatcggagctgcagatgacccagtcccctagctctttaagcgcttccgtgggcgacagagtgaccatcacatgtcgtacctcccagagcatcagctcctatttaaactggtaccagcagaagcccggacagccccccaagctgctgatctactgggcttccactcgtgaaagcggcgtgcccgatcgtttttccggcagcggcagcggcaccgactttactttaaccatctcctctttacagcccgaggatagcgccacctactactgccagcagagctacgacatcccctacacattcggccaaggtaccaagctggaaatcaaacaccaccaccaccaccactga

SEQ ID NO: 48 - DNA, 747 bp, Artificial Sequence
  Synthetic
gagctgcagatgacccagtcccctagctctttaagcgcttccgtgggcgacagagtgaccatcacatgtcgtacctcccagagcatcagctcctatttaaactggtaccagcagaagcccggacagccccccaagctgctgatctactgggcttccactcgtgaaagcggcgtgcccgatcgtttttccggcagcggcagcggcaccgactttactttaaccatctcctctttacagcccgaggatagcgccacctactactgccagcagagctacgacatcccctacacattcggccaaggtaccaagctggaaatcaaaggcggcggcggcagcggcggcggcggctccggcggaggaggctccgaagtgcagctgctggagagcggaggcggagtggtgcaacccggtcgttctttaaggctgagctgcgctgccagcggcttcaccttcagcagctatggcatgcactgggtgagacaagctcccggaaaaggtttagagtgggtggccgtgatctcctacgacggcagcaacaagtactacgccgacagcgtgaagggtcgtttcaccatctctcgtgacaactccaagaacactttatacctccagatgaactctttaagggccgaggacaccgccgtgtactactgtgccaaggacatgggctggggcagcggatggaggccctactactactacggcatggacgtgtggggccaaggtacaaccgtgaccgtgtccagc

SEQ ID NO: 49 - DNA, 681 bp, Artificial Sequence
  Synthetic
aggctgcagatgacccagtcccctagctctttaagcgcttccgtgggcgacagagtgaccatcacatgtcgtacctcccagagcatcagctcctatttaaactggtaccaggataagcccggacagccccccaagctgctgatctactgggcttccactcgtgaaagcggcgtgcccgatcgtttttccggcagcggcagcggcaccgactttactttaaccatctcctctttacagcccgaggatagcgccacctactactgccagcagagctacgacatcccctacacattcggccaaggtaccaagctggaaatcaaaaccgtggcagcaccatccgtgttcatctttcccccttctgacgagcagctgaagtctggcacagccagcgtggtgtgctacctgaacaacttctaccccagggaggccaaggtgcagtggaaggtggataacgccctgcagtccggcaattctcaggagagcgtgaccgagcaggactccaaggattctacatacagcctgtggtccaccctgacactgtccaaggccgactacgagaagcacaagctgtatgcatgcgaggtgacccaccagggcctgtcctctcccgtgacaaagagcttcaataggggagagtgtggaggaggatcctacccttatgacgtgccagattatgcctaa

SEQ ID NO: 50 - DNA, 1374 bp, Artificial Sequence
  Synthetic
gaagtgcagctgctggagagcggaggcggagtggtgcaacccggtcgttctttaaggctgagctgcgctgccagcggcttcaccttcagcagctatggcatgcactgggtgagaaaggctcccggaaaaggtttagagtgggtggccgtgatctcctacgacggcagcaacaagtactacgccgacagcgtgaagggtgagttcaccatctctcgtgacaactccaagaacactttatacctccagatgaactctttaagggccgaggacaccgccgtgtactactgtgccaaggacatgggctggggcagcggatggaggccctactactactacggcatggacgtgtggggccaaggtacaaccgtgaccgtgtccagcgcctctacaaagggaccaagcgtgtttccactggcaccctcctctaagagcacctccggaggaacagccgccctgggctgtctggtgaaggactatttcccagagcccgtgaccgtgtcctggaactctggcgccctgacctccggagtggcaacaggaccagccgtgctgcagagctccggcctgtacagcctgtctagcgtggtgaccgtgccctcctctagcctgggcacccagacatatatctgcaacgtgaatcacaagccaagcaatacaaaggtcgacaagaaggtggagcccaagtcctgtgataagacccacacatgccccccttgtcctgcaccagagctgctgggaggaccaagcgtgttcctgtttccacccaagcctaaggacaccctgatgatctctaggacccccgaggtgacatgcgtggtggtggacgtgagccacgaggatcctgaggtgaagtttaactggtacgtggatggcgtggaggtgcacaatgccaagaccaagccccgggaggagcagtacaactccacctatagagtggtgtctgtgctgacagtgctgcaccaggactggctgaacggcaaggagtataagtgcaaggtgtccaataaggccctgcccgcccctatcgagaagaccatctctaaggccaagggccagcctagggagccacaggtgtacacactgcctccatcccgcaaggagctgaccaagaaccaggtgtctctgacatgtctggtgaagggcttctatccttctgatatcgccgtggagtgggagagcaatggccagccagagaacaattacaagaccacaccccctgtgctgaagagcgacggctccttctttctgtatagcaagctgaccgtggataagtccagatggcagcagggcaacgtgttttcttgtagcgtgatgcacgaggccctgcacaatcactacacacagaagtccctgtctctgagccctggcaagtaa

SEQ ID NO: 51 - DNA, 648 bp, Artificial Sequence
  Synthetic
gatattcagatgacccagagcccgagcagcctgagcgcaagcgttggtgatcgtgttaccattacctgtaaagcaagccagaccgttagcgcaaatgttgcatggtatcagcagaaaccgggtaaagcaccgaaactgctgatttatctggcaagctatcgttatcgtggtgttccgagccgttttagcggtagcggtagcggtaccgattttaccctgaccattagcagcctgcagccggaagattttgcaacctattattgtcatcagtattatacctatccgctgtttacctttggtcagggtaccaaactggaaattaaacgtactgtggctgcaccatctgtcttcatcttcccgccatctgatgagcagttgaaatctggaactgcctctgttgtgtgcctgctgaataacttctatcccagagaggccaaagtacagtggaaggtggataacgccctccaatcgggtaactcccaggagagtgtcacagagcaggacagcaaggacagcacctacagcctcagcagcaccctgacgctgagcaaagcagactacgagaaacacaaactctacgcctgcgaagtcacccatcagggcctgagctcgcccgtcacaaagagcttcaacaggggagagtgctga

SEQ ID NO: 52 - DNA, 678 bp, Artificial Sequence
  Synthetic
caggttcagctggttcagagcggtagcgaactgaaaaaaccgggtgcaagcgttaaagttagctgtaaagcaagcggttatacctttaccgaatatggtatgaatgtttggcgtcaggcaccgggtcagggtctggaatggatgggttggattaataccaaaagcggtgaagcaacctatgttgaagaatttaaaggtcgttttgtttttagcctggataccagcgttagcaccgcatatctgcagattagcagcctgaaagcagaagataccgcagtttattattgtgcacgttgggatttttatgattatgttgatgaagcaatgtattggggtcagggtaccaccgttaccgttagcagcgcctccaccaagggcccatcggtcttccccctggcaccctcctccaagagcacctctgggggcacagcggccctgggctgcctggtcaaggactacttccccgaaccggtgacggtgtcgtggaactcaggcgccctgaccagcggcgtgcacaccttcccggctgtcctacagtcctcaggactctactccctcagcagcgtggtgaccgtgccctccagcagcttgggcacccagacctacatctgcaacgtgaatcacaagcccagcaacaccaaggtggacaagagagttgagcccaaatcttgtgacaaa

SEQ ID NO: 53 - DNA, 777 bp, Artificial Sequence
  Synthetic
ggcggcggcagcggcggcggccaggttcagctggttcagagcggtagcgaactgaaaaaaccgggtgcaagcgttaaagttagctgtaaagcaagcggttatacctttaccgaatatggtatgaatgtttggcgtcaggcaccgggtcagggtctggaatggatgggttggattaataccaaaagcggtgaagcaacctatgttgaagaatttaaaggtcgttttgtttttagcctggataccagcgttagcaccgcatatctgcagattagcagcctgaaagcagaagataccgcagtttattattgtgcacgttgggatttttatgattatgttgatgaagcaatgtattggggtcagggtaccaccgttaccgttagcagcggtggaggcggttcaggcggaggtggctctggcggtggcggatcggatattcagatgacccagagcccgagcagcctgagcgcaagcgttggtgatcgtgttaccattacctgtaaagcaagccagaccgttagcgcaaatgttgcatggtatcagcagaaaccgggtaaagcaccgaaactgctgatttatctggcaagctatcgttatcgtggtgttccgagccgttttagcggtagcggtagcggtaccgattttaccctgaccattagcagcctgcagccggaagattttgcaacctattattgtcatcagtattatacctatccgctgtttacctttggtcagggtaccaaactggaaattaaacgtcaccaccaccaccaccactga

SEQ ID NO: 54 - DNA, 735 bp, Artificial Sequence
  Synthetic
gatattcagatgacccagagcccgagcagcctgagcgcaagcgttggtgatcgtgttaccattacctgtaaagcaagccagaccgttagcgcaaatgttgcatggtatcagcagaaaccgggtaaagcaccgaaactgctgatttatctggcaagctatcgttatcgtggtgttccgagccgttttagcggtagcggtagcggtaccgattttaccctgaccattagcagcctgcagccggaagattttgcaacctattattgtcatcagtattatacctatccgctgtttacctttggtcagggtaccaaactggaaattaaacgtggtggaggcggttcaggcggaggtggctctggcggtggcggatcgcaggttcagctggttcagagcggtagcgaactgaaaaaaccgggtgcaagcgttaaagttagctgtaaagcaagcggttatacctttaccgaatatggtatgaatgtttggcgtcaggcaccgggtcagggtctggaatggatgggttggattaataccaaaagcggtgaagcaacctatgttgaagaatttaaaggtcgttttgtttttagcctggataccagcgttagcaccgcatatctgcagattagcagcctgaaagcagaagataccgcagtttattattgtgcacgttgggatttttatgattatgttgatgaagcaatgtattggggtcagggtaccaccgttaccgttagcagc

SEQ ID NO: 55 - DNA, 687 bp, Artificial Sequence
  Synthetic
aggattcagatgacccagagcccgagcagcctgagcgcaagcgttggtgatcgtgttaccattacctgtaaagcaagccagaccgttagcgcaaatgttgcatggtatcaggataaaccgggtaaagcaccgaaactgctgatttatctggcaagctatcgttatcgtggtgttccgagccgttttagcggtagcggtagcggtaccgattttaccctgaccattagcagcctgcagccggaagattttgcaacctattattgtcatcagtattatacctatccgctgtttacctttggtcagggtaccaaactggaaattaaacgtaccgtggcagcaccatccgtgttcatctttcccccttctgacgagcagctgaagtctggcacagccagcgtggtgtgctacctgaacaacttctaccccagggaggccaaggtgcagtggaaggtggataacgccctgcagtccggcaattctcaggagagcgtgaccgagcaggactccaaggattctacatacagcctgtggtccaccctgacactgtccaaggccgactacgagaagcacaagctgtatgcatgcgaggtgacccaccagggcctgtcctctcccgtgacaaagagcttcaataggggagagtgtggaggaggatcctacccttatgacgtgccagattatgcctaa

SEQ ID NO: 56 - DNA, 1356 bp, Artificial Sequence
  Synthetic
caggttcagctggttcagagcggtagcgaactgaaaaaaccgggtgcaagcgttaaagttagctgtaaagcaagcggttatacctttaccgaatatggtatgaatgtttggcgtaaggcaccgggtcagggtctggaatggatgggttggattaataccaaaagcggtgaagcaacctatgttgaagaatttaaaggtcgttttgtttttagcctggataccagcgttagcaccgcatatctgcagattagcagcctgaaagcagaagataccgcagtttattattgtgcacgttgggatttttatgattatgttgatgaagcaatgtattggggtcagggtaccaccgttaccgttagcagcgcctctacaaagggaccaagcgtgtttccactggcaccctcctctaagagcacctccggaggaacagccgccctgggctgtctggtgaaggactatttcccagagcccgtgaccgtgtcctggaactctggcgccctgacctccggagtggcaacaggaccagccgtgctgcagagctccggcctgtacagcctgtctagcgtggtgaccgtgccctcctctagcctgggcacccagacatatatctgcaacgtgaatcacaagccaagcaatacaaaggtcgacaagaaggtggagcccaagtcctgtgataagacccacacatgccccccttgtcctgcaccagagctgctgggaggaccaagcgtgttcctgtttccacccaagcctaaggacaccctgatgatctctaggacccccgaggtgacatgcgtggtggtggacgtgagccacgaggatcctgaggtgaagtttaactggtacgtggatggcgtggaggtgcacaatgccaagaccaagccccgggaggagcagtacaactccacctatagagtggtgtctgtgctgacagtgctgcaccaggactggctgaacggcaaggagtataagtgcaaggtgtccaataaggccctgcccgcccctatcgagaagaccatctctaaggccaagggccagcctagggagccacaggtgtacacactgcctccatcccgcaaggagctgaccaagaaccaggtgtctctgacatgtctggtgaagggcttctatccttctgatatcgccgtggagtgggagagcaatggccagccagagaacaattacaagaccacaccccctgtgctgaagagcgacggctccttctttctgtatagcaagctgaccgtggataagtccagatggcagcagggcaacgtgttttcttgtagcgtgatgcacgaggccctgcacaatcactacacacagaagtccctgtctctgagccctggcaagtaa

SEQ ID NO: 57 - DNA, 654 bp, Artificial Sequence
  Synthetic
gatattcagatgacccagagcccgagcagcctgagcgcgagcgtgggcgatcgcgtgaccattacctgccaggcgagccagagcattagcagcagctatctgagctggtatcagcagaaaccgggcaaagcgccgaaactgctgatttatgcggtgagctatctggcgagcggcgtgccgagccgctttagcggcagcggcagcggcaccgatttcaccctgaccattagcagcctgcagccggaagattttgcgacctattattgccagagcggctattatagcgcgggcgatctgacctttggccagggcaccaaagtggaaattaaacgcactgtggctgcaccatctgtcttcatcttcccgccatctgatgagcagttgaaatctggaactgcctctgttgtgtgcctgctgaataacttctatcccagagaggccaaagtacagtggaaggtggataacgccctccaatcgggtaactcccaggagagtgtcacagagcaggacagcaaggacagcacctacagcctcagcagcaccctgacgctgagcaaagcagactacgagaaacacaaactctacgcctgcgaagtcacccatcagggcctgagctcgcccgtcacaaagagcttcaacaggggagagtgctga

SEQ ID NO: 58 - DNA, 660 bp, Artificial Sequence
  Synthetic
gaagtgcagctggtggaaagcggcggcggcctggtgcagccgggcggcagcctgcgcctgagctgcgcggcgagcggctttagcctgagcaactattatattaactgggtgcgccaggcgccgggcaaaggcctggaatgggtggcgattattttttgcgcgggcaacgcgtataacgcgagctgggcgaaaggccgctttaccattagccgcgatgatagcaaaaacaccctgtatctgcagatgaacagcctgcgcgcggaagataccgcggtgtattattgcgcgcgcggctggcaggcgctggtgaactggggccagggcaccctggtgaccgtgagcagcgcctccaccaagggcccatcggtcttccccctggcaccctcctccaagagcacctctgggggcacagcggccctgggctgcctggtcaaggactacttccccgaaccggtgacggtgtcgtggaactcaggcgccctgaccagcggcgtgcacaccttcccggctgtcctacagtcctcaggactctactccctcagcagcgtggtgaccgtgccctccagcagcttgggcacccagacctacatctgcaacgtgaatcacaagcccagcaacaccaaggtggacaagagagttgagcccaaatcttgtgacaaa

SEQ ID NO: 59 - DNA, 765 bp, Artificial Sequence
  Synthetic
ggcggcggcagcggcggcggcgaagtgcagctggtggaaagcggcggcggcctggtgcagccgggcggcagcctgcgcctgagctgcgcggcgagcggctttagcctgagcaactattatattaactgggtgcgccaggcgccgggcaaaggcctggaatgggtggcgattattttttgcgcgggcaacgcgtataacgcgagctgggcgaaaggccgctttaccattagccgcgatgatagcaaaaacaccctgtatctgcagatgaacagcctgcgcgcggaagataccgcggtgtattattgcgcgcgcggctggcaggcgctggtgaactggggccagggcaccctggtgaccgtgagcagcggcggcggcggcagcggcggcggcggcagcggcggcggcggcagcgatattcagatgacccagagcccgagcagcctgagcgcgagcgtgggcgatcgcgtgaccattacctgccaggcgagccagagcattagcagcagctatctgagctggtatcagcagaaaccgggcaaagcgccgaaactgctgatttatgcggtgagctatctggcgagcggcgtgccgagccgctttagcggcagcggcagcggcaccgatttcaccctgaccattagcagcctgcagccggaagattttgcgacctattattgccagagcggctattatagcgcgggcgatctgacctttggccagggcaccaaagtggaaattaaacgccaccaccaccaccaccactga

SEQ ID NO: 60 - DNA, 723 bp, Artificial Sequence
  Synthetic
gatattcagatgacccagagcccgagcagcctgagcgcgagcgtgggcgatcgcgtgaccattacctgccaggcgagccagagcattagcagcagctatctgagctggtatcagcagaaaccgggcaaagcgccgaaactgctgatttatgcggtgagctatctggcgagcggcgtgccgagccgctttagcggcagcggcagcggcaccgatttcaccctgaccattagcagcctgcagccggaagattttgcgacctattattgccagagcggctattatagcgcgggcgatctgacctttggccagggcaccaaagtggaaattaaacgcggtggaggcggttcaggcggaggtggctctggcggtggcggatcggaagtgcagctggtggaaagcggcggcggcctggtgcagccgggcggcagcctgcgcctgagctgcgcggcgagcggctttagcctgagcaactattatattaactgggtgcgccaggcgccgggcaaaggcctggaatgggtggcgattattttttgcgcgggcaacgcgtataacgcgagctgggcgaaaggccgctttaccattagccgcgatgatagcaaaaacaccctgtatctgcagatgaacagcctgcgcgcggaagataccgcggtgtattattgcgcgcgcggctggcaggcgctggtgaactggggccagggcaccctggtgaccgtgagcagc

SEQ ID NO: 61 - DNA, 693 bp, Artificial Sequence
  Synthetic
aggattcagatgacccagagcccgagcagcctgagcgcgagcgtgggcgatcgcgtgaccattacctgccaggcgagccagagcattagcagcagctatctgagctggtatcaggataaaccgggcaaagcgccgaaactgctgatttatgcggtgagctatctggcgagcggcgtgccgagccgctttagcggcagcggcagcggcaccgatttcaccctgaccattagcagcctgcagccggaagattttgcgacctattattgccagagcggctattatagcgcgggcgatctgacctttggccagggcaccaaagtggaaattaaacgcaccgtggcagcaccatccgtgttcatctttcccccttctgacgagcagctgaagtctggcacagccagcgtggtgtgctacctgaacaacttctaccccagggaggccaaggtgcagtggaaggtggataacgccctgcagtccggcaattctcaggagagcgtgaccgagcaggactccaaggattctacatacagcctgtggtccaccctgacactgtccaaggccgactacgagaagcacaagctgtatgcatgcgaggtgacccaccagggcctgtcctctcccgtgacaaagagcttcaataggggagagtgtggaggaggatcctacccttatgacgtgccagattatgcctaa

SEQ ID NO: 62 - DNA, 1338 bp, Artificial Sequence
  Synthetic
gaagtgcagctggtggaaagcggcggcggcctggtgcagccgggcggcagcctgcgcctgagctgcgcggcgagcggctttagcctgagcaactattatattaactgggtgcgcaaggcgccgggcaaaggcctggaatgggtggcgattattttttgcgcgggcaacgcgtataacgcgagctgggcgaaaggcgagtttaccattagccgcgatgatagcaaaaacaccctgtatctgcagatgaacagcctgcgcgcggaagataccgcggtgtattattgcgcgcgcggctggcaggcgctggtgaactggggccagggcaccctggtgaccgtgagcagcgcctctacaaagggaccaagcgtgtttccactggcaccctcctctaagagcacctccggaggaacagccgccctgggctgtctggtgaaggactatttcccagagcccgtgaccgtgtcctggaactctggcgccctgacctccggagtggcaacaggaccagccgtgctgcagagctccggcctgtacagcctgtctagcgtggtgaccgtgccctcctctagcctgggcacccagacatatatctgcaacgtgaatcacaagccaagcaatacaaaggtcgacaagaaggtggagcccaagtcctgtgataagacccacacatgccccccttgtcctgcaccagagctgctgggaggaccaagcgtgttcctgtttccacccaagcctaaggacaccctgatgatctctaggacccccgaggtgacatgcgtggtggtggacgtgagccacgaggatcctgaggtgaagtttaactggtacgtggatggcgtggaggtgcacaatgccaagaccaagccccgggaggagcagtacaactccacctatagagtggtgtctgtgctgacagtgctgcaccaggactggctgaacggcaaggagtataagtgcaaggtgtccaataaggccctgcccgcccctatcgagaagaccatctctaaggccaagggccagcctagggagccacaggtgtacacactgcctccatcccgcaaggagctgaccaagaaccaggtgtctctgacatgtctggtgaagggcttctatccttctgatatcgccgtggagtgggagagcaatggccagccagagaacaattacaagaccacaccccctgtgctgaagagcgacggctccttctttctgtatagcaagctgaccgtggataagtccagatggcagcagggcaacgtgttttcttgtagcgtgatgcacgaggccctgcacaatcactacacacagaagtccctgtctctgagccctggcaagtaa

SEQ ID NO: 63 - protein, 21 aa, Artificial Sequence
  Synthetic
METDTLLLWVLLLWVPGSTGD

SEQ ID NO: 64 - protein, 214 aa, Artificial Sequence
  Synthetic
DIVMTQSPSSLSASVGDRVTITCKASQDVGTAVDWYQQKPGKAPKLLIYWASTRHTGVPDRFTGSGSGTDFTLTISSLQPEDFADYFCQQYNSYPLTFGGGTKLEIKRTVAAPSVFIFPPSDEQLKSGTASVVCLLNNFYPREAKVQWKVDNALQSGNSQESVTEQDSKDSTYSLSSTLTLSKADYEKHKLYACEVTHQGLSSPVTKSFNRGEC

SEQ ID NO: 65 - protein, 220 aa, Artificial Sequence
  Synthetic
EVQLVQSGAEVKKPGASVKISCKTSGYTFTEYTIHWVKQASGKGLEWIGNINPNNGGTTYNQKFEDRATLTVDKSTSTAYMELSSLRSEDTAVYYCAAGWNFDYWGQGTTVTVSSASTKGPSVFPLAPSSKSTSGGTAALGCLVKDYFPEPVTVSWNSGALTSGVHTFPAVLQSSGLYSLSSVVTVPSSSLGTQTYICNVNHKPSNTKVDKRVEPKSCDK

SEQ ID NO: 66 - protein, 257 aa, Artificial Sequence
  Synthetic
GGGSGGGDIKLQQSGAELARPGASVKMSCKTSGYTFTRYTMHWVKQRPGQGLEWIGYINPSRGYTNYNQKFKDKATLTTDKSSSTAYMQLSSLTSEDSAVYYCARYYDDHYCLDYWGQGTTLTVSSVEGGSGGSGGSGGSGGVDDIQLTQSPAIMSASPGEKVTMTCRASSSVSYMNWYQQKSGTSPKRWIYDTSKVASGVPYRFSGSGSGTSYSLTISSMEAEDAATYYCQQWSSNPLTFGAGTKLELKRHHHHHH

SEQ ID NO: 67 - protein, 213 aa, Artificial Sequence
  Synthetic
DIQLTQSPAIMSASPGEKVTMTCRASSSVSYMNWYQQKSGTSPKRWIYDTSKVASGVPYRFSGSGSGTSYSLTISSMEAEDAATYYCQQWSSNPLTFGAGTKLELKRTVAAPSVFIFPPSDEQLKSGTASVVCLLNNFYPREAKVQWKVDNALQSGNSQESVTEQDSKDSTYSLSSTLTLSKADYEKHKLYACEVTHQGLSSPVTKSFNRGEC

SEQ ID NO: 68 - protein, 217 aa, Artificial Sequence
  Synthetic
DIKLQQSGAELARPGASVKMSCKTSGYTFTRYTMHWVKQRPGQGLEWIGYINPSRGYTNYNQKFKDKATLTTDKSSSTAYMQLSSLTSEDSAVYYCARYYDDHYCLDYWGQGTTLTVSSASTKGPSVFPLAPCSRSTSESTAALGCLVKDYFPEPVTVSWNSGALTSGVHTFPAVLQSSGLYSLSSVVTVPSSNFGTQTYTCNVDHKPSNTKVDKTV

SEQ ID NO: 69 - protein, 252 aa, Artificial Sequence
  Synthetic
GGGSGGGEVQLVQSGAEVKKPGASVKISCKTSGYTFTEYTIHWVKQASGKGLEWIGNINPNNGGTTYNQKFEDRATLTVDKSTSTAYMELSSLRSEDTAVYYCAAGWNFDYWGQGTTVTVSSAGGGGSGGGGSGGGGSDIVMTQSPSSLSASVGDRVTITCKASQDVGTAVDWYQQKPGKAPKLLIYWASTRHTGVPDRFTGSGSGTDFTLTISSLQPEDFADYFCQQYNSYPLTFGGGTKLEIKRHHHHHH

SEQ ID NO: 70 - protein, 239 aa, Artificial Sequence
  Synthetic
DIVMTQSPSSLSASVGDRVTITCKASQDVGTAVDWYQQKPGKAPKLLIYWASTRHTGVPDRFTGSGSGTDFTLTISSLQPEDFADYFCQQYNSYPLTFGGGTKLEIKRGGGGSGGGGSGGGGSEVQLVQSGAEVKKPGASVKISCKTSGYTFTEYTIHWVKQASGKGLEWIGNINPNNGGTTYNQKFEDRATLTVDKSTSTAYMELSSLRSEDTAVYYCAAGWNFDYWGQGTTVTVSSA

SEQ ID NO: 71 - protein, 223 aa, Artificial Sequence
  Synthetic
DIQLTQSPAIMSASPGEKVTMTCRASSSVSYMNWYQRKSGTSPKRWIYDTSKVASGVPYRFSGSGSGTSYSLTISSMEAEDAATYYCQQWSSNPLTFGAGTKLELKRTVAAPSVFIFPPSDEQLKSGTASVVCLLNNFYPREAKVQWKVDNALQSGNSQESVTEQDSKDSTYSLSSTLTLSKADYEKHKLYACEVTHQGLSSPVTKSFNRGECGGGSHHHHHH

SEQ ID NO: 72 - protein, 449 aa, Artificial Sequence
  Synthetic
DIKLQQSGAELARPGASVKMSCKTSGYTFTRYTMHWVKYRPGQGLEWIGYINPSRGYTNYNQKFKDKATLTTDKSSSTAYMQLSSLTSEDSAVYYCARYYDDHYCLDYWGQGTTLTVSSASTKGPSVFPLAPSSKSTSGGTAALGCLVKDYFPEPVTVSWNSGALTSGVHTFPAVLQSSGLYSLSSVVTVPSSSLGTQTYICNVNHKPSNTKVDKKVEPKSCDKTHTCPPCPAPELLGGPSVFLFPPKPKDTLMISRTPEVTCVVVDVSHEDPEVKFNWYVDGVEVHNAKTKPREEQYNSTYRVVSVLTVLHQDWLNGKEYKCKVSNKALPAPIEKTISKAKGQPREPQVYTLPPSRDELTKNQVSLTCLVKGFYPSDIAVEWESNGQPENNYDTTPPVLDSDGSFFLYSDLTVDKSRWQQGNVFSCSVMHEALHNHYTQKSLSLSPGK

SEQ ID NO: 73 - protein, 227 aa, Artificial Sequence
  Synthetic
RIVMTQSPSSLSASVGDRVTITCKASQDVGTAVDWYQDKPGKAPKLLIYWASTRHTGVPDRFTGSGSGTDFTLTISSLQPEDFADYFCQQYNSYPLTFGGGTKLEIKRTVAAPSVFIFPPSDEQLKSGTASVVCYLNNFYPREAKVQWKVDNALQSGNSQESVTEQDSKDSTYSLWSTLTLSKADYEKHKLYACEVTHQGLSSPVTKSFNRGECGGGSYPYDVPDYA

SEQ ID NO: 74 - protein, 445 aa, Artificial Sequence
  Synthetic
EVQLVQSGAEVKKPGASVKISCKTSGYTFTEYTIHWVKKASGKGLEWIGNINPNNGGTTYNQEFEDRATLTVDKSTSTAYMELSSLRSEDTAVYYCAAGWNFDYWGQGTTVTVSSASTKGPSVFPLAPSSKSTSGGTAALGCLVKDYFPEPVTVSWNSGALTSGVATGPAVLQSSGLYSLSSVVTVPSSSLGTQTYICNVNHKPSNTKVDKKVEPKSCDKTHTCPPCPAPELLGGPSVFLFPPKPKDTLMISRTPEVTCVVVDVSHEDPEVKFNWYVDGVEVHNAKTKPREEQYNSTYRVVSVLTVLHQDWLNGKEYKCKVSNKALPAPIEKTISKAKGQPREPQVYTLPPSRKELTKNQVSLTCLVKGFYPSDIAVEWESNGQPENNYKTTPPVLKSDGSFFLYSKLTVDKSRWQQGNVFSCSVMHEALHNHYTQKSLSLSPGK

SEQ ID NO: 75 - protein, 214 aa, Artificial Sequence
  Synthetic
DILLTQSPVILSVSPGERVSFSCRASQSIGTNIHWYQQRTNGSPRLLIKYASESISGIPSRFSGSGSGTDFTLSINSVESEDIADYYCQQNNNWPTTFGAGTKLELKRTVAAPSVFIFPPSDEQLKSGTASVVCLLNNFYPREAKVQWKVDNALQSGNSQESVTEQDSKDSTYSLSSTLTLSKADYEKHKLYACEVTHQGLSSPVTKSFNRGEC

SEQ ID NO: 76 - protein, 224 aa, Artificial Sequence
  Synthetic
QVQLKQSGPGLVQPSQSLSITCTVSGFSLTNYGVHWVRQSPGKGLEWLGVIWSGGNTDYNTPFTSRLSINKDNSKSQVFFKMNSLQSNDTAIYYCARALTYYDYEFAYWGQGTLVTVSAASTKGPSVFPLAPSSKSTSGGTAALGCLVKDYFPEPVTVSWNSGALTSGVHTFPAVLQSSGLYSLSSVVTVPSSSLGTQTYICNVNHKPSNTKVDKRVEPKSCDK

SEQ ID NO: 77 - protein, 255 aa, Artificial Sequence
  Synthetic
GGGSGGGQVQLKQSGPGLVQPSQSLSITCTVSGFSLTNYGVHWVRQSPGKGLEWLGVIWSGGNTDYNTPFTSRLSINKDNSKSQVFFKMNSLQSNDTAIYYCARALTYYDYEFAYWGQGTLVTVSAGGGGSGGGGSGGGGSDILLTQSPVILSVSPGERVSFSCRASQSIGTNIHWYQQRTNGSPRLLIKYASESISGIPSRFSGSGSGTDFTLSINSVESEDIADYYCQQNNNWPTTFGAGTKLELKRHHHHHH

SEQ ID NO: 78 - protein, 242 aa, Artificial Sequence
  Synthetic
DILLTQSPVILSVSPGERVSFSCRASQSIGTNIHWYQQRTNGSPRLLIKYASESISGIPSRFSGSGSGTDFTLSINSVESEDIADYYCQQNNNWPTTFGAGTKLELKRGGGGSGGGGSGGGGSQVQLKQSGPGLVQPSQSLSITCTVSGFSLTNYGVHWVRQSPGKGLEWLGVIWSGGNTDYNTPFTSRLSINKDNSKSQVFFKMNSLQSNDTAIYYCARALTYYDYEFAYWGQGTLVTVSA

SEQ ID NO: 79 - protein, 254 aa, Artificial Sequence
  Synthetic
GGGSDIKLQQSGAELARPGASVKMSCKTSGYTFTRYTMHWVKQRPGQGLEWIGYINPSRGYTNYNQKFKDKATLTTDKSSSTAYMQLSSLTSEDSAVYYCARYYDDHYCLDYWGQGTTLTVSSVEGGSGGSGGSGGSGGVDDIQLTQSPAIMSASPGEKVTMTCRASSSVSYMNWYQQKSGTSPKRWIYDTSKVASGVPYRFSGSGSGTSYSLTISSMEAEDAATYYCQQWSSNPLTFGAGTKLELKRHHHHHH

SEQ ID NO: 80 - protein, 227 aa, Artificial Sequence
  Synthetic
RILLTQSPVILSVSPGERVSFSCRASQSIGTNIHWYQDRTNGSPRLLIKYASESISGIPSRFSGSGSGTDFTLSINSVESEDIADYYCQQNNNWPTTFGAGTKLELKRTVAAPSVFIFPPSDEQLKSGTASVVCYLNNFYPREAKVQWKVDNALQSGNSQESVTEQDSKDSTYSLWSTLTLSKADYEKHKLYACEVTHQGLSSPVTKSFNRGECGGGSYPYDVPDYA

SEQ ID NO: 81 - protein, 449 aa, Artificial Sequence
  Synthetic
QVQLKQSGPGLVQPSQSLSITCTVSGFSLTNYGVHWVRKSPGKGLEWLGVIWSGGNTDYNTEFTSRLSINKDNSKSQVFFKMNSLQSNDTAIYYCARALTYYDYEFAYWGQGTLVTVSAASTKGPSVFPLAPSSKSTSGGTAALGCLVKDYFPEPVTVSWNSGALTSGVATGPAVLQSSGLYSLSSVVTVPSSSLGTQTYICNVNHKPSNTKVDKKVEPKSCDKTHTCPPCPAPELLGGPSVFLFPPKPKDTLMISRTPEVTCVVVDVSHEDPEVKFNWYVDGVEVHNAKTKPREEQYNSTYRVVSVLTVLHQDWLNGKEYKCKVSNKALPAPIEKTISKAKGQPREPQVYTLPPSRKELTKNQVSLTCLVKGFYPSDIAVEWESNGQPENNYKTTPPVLKSDGSFFLYSKLTVDKSRWQQGNVFSCSVMHEALHNHYTQKSLSLSPGK

SEQ ID NO: 82 - protein, 214 aa, Artificial Sequence
  Synthetic
DIQMTQSPSSLSASVGDRVTITCRASQDVSTAVAWYQQKPGKAPKLLIYSASFLYSGVPSRFSGSGSGTDFTLTISSLQPEDFATYYCQQYLYHPATFGQGTKVEIKRTVAAPSVFIFPPSDEQLKSGTASVVCLLNNFYPREAKVQWKVDNALQSGNSQESVTEQDSKDSTYSLSSTLTLSKADYEKHKLYACEVTHQGLSSPVTKSFNRGEC

SEQ ID NO: 83 - protein, 223 aa, Artificial Sequence
  Synthetic
EVQLVESGGGLVQPGGSLRLSCAASGFTFSDSWIHWVRQAPGKGLEWVAWISPYGGSTYYADSVKGRFTISADTSKNTAYLQMNSLRAEDTAVYYCARRHWPGGFDYWGQGTLVTVSAASTKGPSVFPLAPSSKSTSGGTAALGCLVKDYFPEPVTVSWNSGALTSGVHTFPAVLQSSGLYSLSSVVTVPSSSLGTQTYICNVNHKPSNTKVDKRVEPKSCDK

SEQ ID NO: 84 - protein, 257 aa, Artificial Sequence
  Synthetic
GGGSGGGEVQLVESGGGLVQPGGSLRLSCAASGFTFSDSWIHWVRQAPGKGLEWVAWISPYGGSTYYADSVKGRFTISADTSKNTAYLQMNSLRAEDTAVYYCARRHWPGGFDYWGQGTLVTVSAVEGGSGGSGGSGGSGGVDDIQMTQSPSSLSASVGDRVTITCRASQDVSTAVAWYQQKPGKAPKLLIYSASFLYSGVPSRFSGSGSGTDFTLTISSLQPEDFATYYCQQYLYHPATFGQGTKVEIKRHHHHHH

SEQ ID NO: 85 - protein, 241 aa, Artificial Sequence
  Synthetic
DIQMTQSPSSLSASVGDRVTITCRASQDVSTAVAWYQQKPGKAPKLLIYSASFLYSGVPSRFSGSGSGTDFTLTISSLQPEDFATYYCQQYLYHPATFGQGTKVEIKRGGGGSGGGGSGGGGSEVQLVESGGGLVQPGGSLRLSCAASGFTFSDSWIHWVRQAPGKGLEWVAWISPYGGSTYYADSVKGRFTISADTSKNTAYLQMNSLRAEDTAVYYCARRHWPGGFDYWGQGTLVTVSA

SEQ ID NO: 86 - protein, 227 aa, Artificial Sequence
  Synthetic
RIQMTQSPSSLSASVGDRVTITCRASQDVSTAVAWYQDKPGKAPKLLIYSASFLYSGVPSRFSGSGSGTDFTLTISSLQPEDFATYYCQQYLYHPATFGQGTKVEIKRTVAAPSVFIFPPSDEQLKSGTASVVCYLNNFYPREAKVQWKVDNALQSGNSQESVTEQDSKDSTYSLWSTLTLSKADYEKHKLYACEVTHQGLSSPVTKSFNRGECGGGSYPYDVPDYA

SEQ ID NO: 87 - protein, 448 aa, Artificial Sequence
  Synthetic
EVQLVESGGGLVQPGGSLRLSCAASGFTFSDSWIHWVRKAPGKGLEWVAWISPYGGSTYYADSVKGEFTISADTSKNTAYLQMNSLRAEDTAVYYCARRHWPGGFDYWGQGTLVTVSAASTKGPSVFPLAPSSKSTSGGTAALGCLVKDYFPEPVTVSWNSGALTSGVATGPAVLQSSGLYSLSSVVTVPSSSLGTQTYICNVNHKPSNTKVDKKVEPKSCDKTHTCPPCPAPELLGGPSVFLFPPKPKDTLMISRTPEVTCVVVDVSHEDPEVKFNWYVDGVEVHNAKTKPREEQYNSTYRVVSVLTVLHQDWLNGKEYKCKVSNKALPAPIEKTISKAKGQPREPQVYTLPPSRKELTKNQVSLTCLVKGFYPSDIAVEWESNGQPENNYKTTPPVLKSDGSFFLYSKLTVDKSRWQQGNVFSCSVMHEALHNHYTQKSLSLSPGK

SEQ ID NO: 88 - protein, 214 aa, Artificial Sequence
  Synthetic
DIQMTQSPSSLSASVGDRVTITCRASQDVNTAVAWYQQKPGKAPKLLIYSASFLYSGVPSRFSGSRSGTDFTLTISSLQPEDFATYYCQQHYTTPPTFGQGTKVEIKRTVAAPSVFIFPPSDEQLKSGTASVVCLLNNFYPREAKVQWKVDNALQSGNSQESVTEQDSKDSTYSLSSTLTLSKADYEKHKLYACEVTHQGLSSPVTKSFNRGEC

SEQ ID NO: 89 - protein, 225 aa, Artificial Sequence
  Synthetic
EVQLVESGGGLVQPGGSLRLSCAASGFNIKDTYIHWVRQAPGKGLEWVARIYPTNGYTRYADSVKGRFTISADTSKNTAYLQMNSLRAEDTAVYYCSRWGGDGFYAMDYWGQGTLVTVSSASTKGPSVFPLAPSSKSTSGGTAALGCLVKDYFPEPVTVSWNSGALTSGVHTFPAVLQSSGLYSLSSVVTVPSSSLGTQTYICNVNHKPSNTKVDKRVEPKSCDK

SEQ ID NO: 90 - protein, 256 aa, Artificial Sequence
  Synthetic
GGGSGGGEVQLVESGGGLVQPGGSLRLSCAASGFNIKDTYIHWVRQAPGKGLEWVARIYPTNGYTRYADSVKGRFTISADTSKNTAYLQMNSLRAEDTAVYYCSRWGGDGFYAMDYWGQGTLVTVSSGGGGSGGGGSGGGGSDIQMTQSPSSLSASVGDRVTITCRASQDVNTAVAWYQQKPGKAPKLLIYSASFLYSGVPSRFSGSRSGTDFTLTISSLQPEDFATYYCQQHYTTPPTFGQGTKVEIKRHHHHHH

SEQ ID NO: 91 - protein, 243 aa, Artificial Sequence
  Synthetic
DIQMTQSPSSLSASVGDRVTITCRASQDVNTAVAWYQQKPGKAPKLLIYSASFLYSGVPSRFSGSRSGTDFTLTISSLQPEDFATYYCQQHYTTPPTFGQGTKVEIKRGGGGSGGGGSGGGGSEVQLVESGGGLVQPGGSLRLSCAASGFNIKDTYIHWVRQAPGKGLEWVARIYPTNGYTRYADSVKGRFTISADTSKNTAYLQMNSLRAEDTAVYYCSRWGGDGFYAMDYWGQGTLVTVSS

SEQ ID NO: 92 - protein, 227 aa, Artificial Sequence
  Synthetic
RIQMTQSPSSLSASVGDRVTITCRASQDVNTAVAWYQDKPGKAPKLLIYSASFLYSGVPSRFSGSRSGTDFTLTISSLQPEDFATYYCQQHYTTPPTFGQGTKVEIKRTVAAPSVFIFPPSDEQLKSGTASVVCYLNNFYPREAKVQWKVDNALQSGNSQESVTEQDSKDSTYSLWSTLTLSKADYEKHKLYACEVTHQGLSSPVTKSFNRGECGGGSYPYDVPDYA

SEQ ID NO: 93 - protein, 450 aa, Artificial Sequence
  Synthetic
EVQLVESGGGLVQPGGSLRLSCAASGFNIKDTYIHWVRKAPGKGLEWVARIYPTNGYTRYADSVKGRFTISADTSKNTAYLQMNSLRAEDTAVYYCSRWGGDGFYAMDYWGQGTLVTVSSASTKGPSVFPLAPSSKSTSGGTAALGCLVKDYFPEPVTVSWNSGALTSGVATGPAVLQSSGLYSLSSVVTVPSSSLGTQTYICNVNHKPSNTKVDKKVEPKSCDKTHTCPPCPAPELLGGPSVFLFPPKPKDTLMISRTPEVTCVVVDVSHEDPEVKFNWYVDGVEVHNAKTKPREEQYNSTYRVVSVLTVLHQDWLNGKEYKCKVSNKALPAPIEKTISKAKGQPREPQVYTLPPSRKELTKNQVSLTCLVKGFYPSDIAVEWESNGQPENNYKTTPPVLKSDGSFFLYSKLTVDKSRWQQGNVFSCSVMHEALHNHYTQKSLSLSPGK

SEQ ID NO: 94 - protein, 219 aa, Artificial Sequence
  Synthetic
DIVMTQSPDSLAVSLGERATINCKSSQSLLYSRNQKNYLAWYQQKPGQPPKLLIFWASTRESGVPDRFSGSGFGTDFTLTISSLQAEDVAVYYCQQYFSYPLTFGQGTKVEIKTVAAPSVFIFPPSDEQLKSGTASVVCLLNNFYPREAKVQWKVDNALQSGNSQESVTEQDSKDSTYSLSSTLTLSKADYEKHKLYACEVTHQGLSSPVTKSFNRGEC

SEQ ID NO: 95 - protein, 229 aa, Artificial Sequence
  Synthetic
QVQLVQSGAEVKKPGASVKVSCKTSRYTFTEYTIHWVRQAPGQRLEWIGGINPNNGIPNYNQKFKGRVTITVDTSASTAYMELSSLRSEDTAVYYCARRRIAYGYDEGHAMDYWGQGTLVTVSSASTKGPSVFPLAPSSKSTSGGTAALGCLVKDYFPEPVTVSWNSGALTSGVHTFPAVLQSSGLYSLSSVVTVPSSSLGTQTYICNVNHKPSNTKVDKRVEPKSCDK

SEQ ID NO: 96 - protein, 268 aa, Artificial Sequence
  Synthetic
GGGSGGGQVQLVQSGAEVKKPGASVKVSCKTSRYTFTEYTIHWVRQAPGQRLEWIGGINPNNGIPNYNQKFKGRVTITVDTSASTAYMELSSLRSEDTAVYYCARRRIAYGYDEGHAMDYWGQGTLVTVSSGSTSGSGKPGSGEGSTKGDIVMTQSPDSLAVSLGERATINCKSSQSLLYSRNQKNYLAWYQQKPGQPPKLLIFWASTRESGVPDRFSGSGFGTDFTLTISSLQAEDVAVYYCQQYFSYPLTFGQGTKVEIKHHHHHH

SEQ ID NO: 97 - protein, 252 aa, Artificial Sequence
  Synthetic
DIVMTQSPDSLAVSLGERATINCKSSQSLLYSRNQKNYLAWYQQKPGQPPKLLIFWASTRESGVPDRFSGSGFGTDFTLTISSLQAEDVAVYYCQQYFSYPLTFGQGTKVEIKGGGGSGGGGSGGGGSQVQLVQSGAEVKKPGASVKVSCKTSRYTFTEYTIHWVRQAPGQRLEWIGGINPNNGIPNYNQKFKGRVTITVDTSASTAYMELSSLRSEDTAVYYCARRRIAYGYDEGHAMDYWGQGTLVTVSS

SEQ ID NO: 98 - protein, 232 aa, Artificial Sequence
  Synthetic
RIVMTQSPDSLAVSLGERATINCKSSQSLLYSRNQKNYLAWYQDKPGQPPKLLIFWASTRESGVPDRFSGSGFGTDFTLTISSLQAEDVAVYYCQQYFSYPLTFGQGTKVEIKTVAAPSVFIFPPSDEQLKSGTASVVCYLNNFYPREAKVQWKVDNALQSGNSQESVTEQDSKDSTYSLWSTLTLSKADYEKHKLYACEVTHQGLSSPVTKSFNRGECGGGSYPYDVPDYA

SEQ ID NO: 99 - protein, 454 aa, Artificial Sequence
  Synthetic
QVQLVQSGAEVKKPGASVKVSCKTSRYTFTEYTIHWVRKAPGQRLEWIGGINPNNGIPNYNQRFKGRVTITVDTSASTAYMELSSLRSEDTAVYYCARRRIAYGYDEGHAMDYWGQGTLVTVSSASTKGPSVFPLAPSSKSTSGGTAALGCLVKDYFPEPVTVSWNSGALTSGVATGPAVLQSSGLYSLSSVVTVPSSSLGTQTYICNVNHKPSNTKVDKKVEPKSCDKTHTCPPCPAPELLGGPSVFLFPPKPKDTLMISRTPEVTCVVVDVSHEDPEVKFNWYVDGVEVHNAKTKPREEQYNSTYRVVSVLTVLHQDWLNGKEYKCKVSNKALPAPIEKTISKAKGQPREPQVYTLPPSRKELTKNQVSLTCLVKGFYPSDIAVEWESNGQPENNYKTTPPVLKSDGSFFLYSKLTVDKSRWQQGNVFSCSVMHEALHNHYTQKSLSLSPGK

SEQ ID NO: 100 - protein, 218 aa, Artificial Sequence
  Synthetic
DIQMTQSPSSLSASVGDRVTITCRSTKSLLHSNGITYLYWYQQKPGKAPKLLIYQMSNLASGVPSRFSSSGSGTDFTLTISSLQPEDFATYYCAQNLEIPRTFGQGTKVELKTVAAPSVFIFPPSDEQLKSGTASVVCLLNNFYPREAKVQWKVDNALQSGNSQESVTEQDSKDSTYSLSSTLTLSKADYEKHKLYACEVTHQGLSSPVTKSFNRGEC

SEQ ID NO: 101 - protein, 221 aa, Artificial Sequence
  Synthetic
EVQLVQSGPGLVQPGGSVRISCAASGYTFTNYGMNWVKQAPGKGLEWMGWINTYTGESTYADSFKGRFTFSLDTSASAAYLQINSLRAEDTAVYYCARFAIKGDYWGQGTLLTVSSASTKGPSVFPLAPSSKSTSGGTAALGCLVKDYFPEPVTVSWNSGALTSGVHTFPAVLQSSGLYSLSSVVTVPSSSLGTQTYICNVNHKPSNTKVDKRVEPKSCDK

SEQ ID NO: 102 - protein, 256 aa, Artificial Sequence
  Synthetic
GGGSGGGEVQLVQSGPGLVQPGGSVRISCAASGYTFTNYGMNWVKQAPGKGLEWMGWINTYTGESTYADSFKGRFTFSLDTSASAAYLQINSLRAEDTAVYYCARFAIKGDYWGQGTLLTVSSGGGGSGGGGSGGGGSDIQMTQSPSSLSASVGDRVTITCRSTKSLLHSNGITYLYWYQQKPGKAPKLLIYQMSNLASGVPSRFSSSGSGTDFTLTISSLQPEDFATYYCAQNLEIPRTFGQGTKVELKHHHHHH

SEQ ID NO: 103 - protein, 254 aa, Artificial Sequence
  Synthetic
DIQMTQSPSSLSASVGDRVTITCRSTKSLLHSNGITYLYWYQQKPGKAPKLLIYQMSNLASGVPSRFSSSGSGTDFTLTISSLQPEDFATYYCAQNLEIPRTFGQGTKVELKRATPSHNSHQVPSAGGPTANSGTSGSEVQLVQSGPGLVQPGGSVRISCAASGYTFTNYGMNWVKQAPGKGLEWMGWINTYTGESTYADSFKGRFTFSLDTSASAAYLQINSLRAEDTAVYYCARFAIKGDYWGQGTLLTVSS

SEQ ID NO: 104 - protein, 231 aa, Artificial Sequence
  Synthetic
RIQMTQSPSSLSASVGDRVTITCRSTKSLLHSNGITYLYWYQDKPGKAPKLLIYQMSNLASGVPSRFSSSGSGTDFTLTISSLQPEDFATYYCAQNLEIPRTFGQGTKVELKTVAAPSVFIFPPSDEQLKSGTASVVCYLNNFYPREAKVQWKVDNALQSGNSQESVTEQDSKDSTYSLWSTLTLSKADYEKHKLYACEVTHQGLSSPVTKSFNRGECGGGSYPYDVPDYA

SEQ ID NO: 105 - protein, 446 aa, Artificial Sequence
  Synthetic
EVQLVQSGPGLVQPGGSVRISCAASGYTFTNYGMNWVKKAPGKGLEWMGWINTYTGESTYADSFKGEFTFSLDTSASAAYLQINSLRAEDTAVYYCARFAIKGDYWGQGTLLTVSSASTKGPSVFPLAPSSKSTSGGTAALGCLVKDYFPEPVTVSWNSGALTSGVATGPAVLQSSGLYSLSSVVTVPSSSLGTQTYICNVNHKPSNTKVDKKVEPKSCDKTHTCPPCPAPELLGGPSVFLFPPKPKDTLMISRTPEVTCVVVDVSHEDPEVKFNWYVDGVEVHNAKTKPREEQYNSTYRVVSVLTVLHQDWLNGKEYKCKVSNKALPAPIEKTISKAKGQPREPQVYTLPPSRKELTKNQVSLTCLVKGFYPSDIAVEWESNGQPENNYKTTPPVLKSDGSFFLYSKLTVDKSRWQQGNVFSCSVMHEALHNHYTQKSLSLSPGK

SEQ ID NO: 106 - protein, 213 aa, Artificial Sequence
  Synthetic
ELQMTQSPSSLSASVGDRVTITCRTSQSISSYLNWYQQKPGQPPKLLIYWASTRESGVPDRFSGSGSGTDFTLTISSLQPEDSATYYCQQSYDIPYTFGQGTKLEIKTVAAPSVFIFPPSDEQLKSGTASVVCLLNNFYPREAKVQWKVDNALQSGNSQESVTEQDSKDSTYSLSSTLTLSKADYEKHKLYACEVTHQGLSSPVTKSFNRGEC

SEQ ID NO: 107 - protein, 232 aa, Artificial Sequence
  Synthetic
EVQLLESGGGVVQPGRSLRLSCAASGFTFSSYGMHWVRQAPGKGLEWVAVISYDGSNKYYADSVKGRFTISRDNSKNTLYLQMNSLRAEDTAVYYCAKDMGWGSGWRPYYYYGMDVWGQGTTVTVSSASTKGPSVFPLAPSSKSTSGGTAALGCLVKDYFPEPVTVSWNSGALTSGVHTFPAVLQSSGLYSLSSVVTVPSSSLGTQTYICNVNHKPSNTKVDKRVEPKSCDK

SEQ ID NO: 108 - protein, 262 aa, Artificial Sequence
  Synthetic
GGGSGGGEVQLLESGGGVVQPGRSLRLSCAASGFTFSSYGMHWVRQAPGKGLEWVAVISYDGSNKYYADSVKGRFTISRDNSKNTLYLQMNSLRAEDTAVYYCAKDMGWGSGWRPYYYYGMDVWGQGTTVTVSSGGGGSGGGGSGGGGSELQMTQSPSSLSASVGDRVTITCRTSQSISSYLNWYQQKPGQPPKLLIYWASTRESGVPDRFSGSGSGTDFTLTISSLQPEDSATYYCQQSYDIPYTFGQGTKLEIKHHHHHH

SEQ ID NO: 109 - protein, 249 aa, Artificial Sequence
  Synthetic
ELQMTQSPSSLSASVGDRVTITCRTSQSISSYLNWYQQKPGQPPKLLIYWASTRESGVPDRFSGSGSGTDFTLTISSLQPEDSATYYCQQSYDIPYTFGQGTKLEIKGGGGSGGGGSGGGGSEVQLLESGGGVVQPGRSLRLSCAASGFTFSSYGMHWVRQAPGKGLEWVAVISYDGSNKYYADSVKGRFTISRDNSKNTLYLQMNSLRAEDTAVYYCAKDMGWGSGWRPYYYYGMDVWGQGTTVTVSS

SEQ ID NO: 110 - protein, 226 aa, Artificial Sequence
  Synthetic
RLQMTQSPSSLSASVGDRVTITCRTSQSISSYLNWYQDKPGQPPKLLIYWASTRESGVPDRFSGSGSGTDFTLTISSLQPEDSATYYCQQSYDIPYTFGQGTKLEIKTVAAPSVFIFPPSDEQLKSGTASVVCYLNNFYPREAKVQWKVDNALQSGNSQESVTEQDSKDSTYSLWSTLTLSKADYEKHKLYACEVTHQGLSSPVTKSFNRGECGGGSYPYDVPDYA

SEQ ID NO: 111 - protein, 457 aa, Artificial Sequence
  Synthetic
EVQLLESGGGVVQPGRSLRLSCAASGFTFSSYGMHWVRKAPGKGLEWVAVISYDGSNKYYADSVKGEFTISRDNSKNTLYLQMNSLRAEDTAVYYCAKDMGWGSGWRPYYYYGMDVWGQGTTVTVSSASTKGPSVFPLAPSSKSTSGGTAALGCLVKDYFPEPVTVSWNSGALTSGVATGPAVLQSSGLYSLSSVVTVPSSSLGTQTYICNVNHKPSNTKVDKKVEPKSCDKTHTCPPCPAPELLGGPSVFLFPPKPKDTLMISRTPEVTCVVVDVSHEDPEVKFNWYVDGVEVHNAKTKPREEQYNSTYRVVSVLTVLHQDWLNGKEYKCKVSNKALPAPIEKTISKAKGQPREPQVYTLPPSRKELTKNQVSLTCLVKGFYPSDIAVEWESNGQPENNYKTTPPVLKSDGSFFLYSKLTVDKSRWQQGNVFSCSVMHEALHNHYTQKSLSLSPGK

SEQ ID NO: 112 - protein, 215 aa, Artificial Sequence
  Synthetic
DIQMTQSPSSLSASVGDRVTITCKASQTVSANVAWYQQKPGKAPKLLIYLASYRYRGVPSRFSGSGSGTDFTLTISSLQPEDFATYYCHQYYTYPLFTFGQGTKLEIKRTVAAPSVFIFPPSDEQLKSGTASVVCLLNNFYPREAKVQWKVDNALQSGNSQESVTEQDSKDSTYSLSSTLTLSKADYEKHKLYACEVTHQGLSSPVTKSFNRGEC

SEQ ID NO: 113 - protein, 226 aa, Artificial Sequence
  Synthetic
QVQLVQSGSELKKPGASVKVSCKASGYTFTEYGMNVWRQAPGQGLEWMGWINTKSGEATYVEEFKGRFVFSLDTSVSTAYLQISSLKAEDTAVYYCARWDFYDYVDEAMYWGQGTTVTVSSASTKGPSVFPLAPSSKSTSGGTAALGCLVKDYFPEPVTVSWNSGALTSGVHTFPAVLQSSGLYSLSSVVTVPSSSLGTQTYICNVNHKPSNTKVDKRVEPKSCDK

SEQ ID NO: 114 - protein, 258 aa, Artificial Sequence
  Synthetic
GGGSGGGQVQLVQSGSELKKPGASVKVSCKASGYTFTEYGMNVWRQAPGQGLEWMGWINTKSGEATYVEEFKGRFVFSLDTSVSTAYLQISSLKAEDTAVYYCARWDFYDYVDEAMYWGQGTTVTVSSGGGGSGGGGSGGGGSDIQMTQSPSSLSASVGDRVTITCKASQTVSANVAWYQQKPGKAPKLLIYLASYRYRGVPSRFSGSGSGTDFTLTISSLQPEDFATYYCHQYYTYPLFTFGQGTKLEIKRHHHHHH

SEQ ID NO: 115 - protein, 245 aa, Artificial Sequence
  Synthetic
DIQMTQSPSSLSASVGDRVTITCKASQTVSANVAWYQQKPGKAPKLLIYLASYRYRGVPSRFSGSGSGTDFTLTISSLQPEDFATYYCHQYYTYPLFTFGQGTKLEIKRGGGGSGGGGSGGGGSQVQLVQSGSELKKPGASVKVSCKASGYTFTEYGMNVWRQAPGQGLEWMGWINTKSGEATYVEEFKGRFVFSLDTSVSTAYLQISSLKAEDTAVYYCARWDFYDYVDEAMYWGQGTTVTVSS

SEQ ID NO: 116 - protein, 228 aa, Artificial Sequence
  Synthetic
RIQMTQSPSSLSASVGDRVTITCKASQTVSANVAWYQDKPGKAPKLLIYLASYRYRGVPSRFSGSGSGTDFTLTISSLQPEDFATYYCHQYYTYPLFTFGQGTKLEIKRTVAAPSVFIFPPSDEQLKSGTASVVCYLNNFYPREAKVQWKVDNALQSGNSQESVTEQDSKDSTYSLWSTLTLSKADYEKHKLYACEVTHQGLSSPVTKSFNRGECGGGSYPYDVPDYA

SEQ ID NO: 117 - protein, 451 aa, Artificial Sequence
  Synthetic
QVQLVQSGSELKKPGASVKVSCKASGYTFTEYGMNVWRKAPGQGLEWMGWINTKSGEATYVEEFKGRFVFSLDTSVSTAYLQISSLKAEDTAVYYCARWDFYDYVDEAMYWGQGTTVTVSSASTKGPSVFPLAPSSKSTSGGTAALGCLVKDYFPEPVTVSWNSGALTSGVATGPAVLQSSGLYSLSSVVTVPSSSLGTQTYICNVNHKPSNTKVDKKVEPKSCDKTHTCPPCPAPELLGGPSVFLFPPKPKDTLMISRTPEVTCVVVDVSHEDPEVKFNWYVDGVEVHNAKTKPREEQYNSTYRVVSVLTVLHQDWLNGKEYKCKVSNKALPAPIEKTISKAKGQPREPQVYTLPPSRKELTKNQVSLTCLVKGFYPSDIAVEWESNGQPENNYKTTPPVLKSDGSFFLYSKLTVDKSRWQQGNVFSCSVMHEALHNHYTQKSLSLSPGK

SEQ ID NO: 118 - protein, 217 aa, Artificial Sequence
  Synthetic
DIQMTQSPSSLSASVGDRVTITCQASQSISSSYLSWYQQKPGKAPKLLIYAVSYLASGVPSRFSGSGSGTDFTLTISSLQPEDFATYYCQSGYYSAGDLTFGQGTKVEIKRTVAAPSVFIFPPSDEQLKSGTASVVCLLNNFYPREAKVQWKVDNALQSGNSQESVTEQDSKDSTYSLSSTLTLSKADYEKHKLYACEVTHQGLSSPVTKSFNRGEC

SEQ ID NO: 119 - protein, 220 aa, Artificial Sequence
  Synthetic
EVQLVESGGGLVQPGGSLRLSCAASGFSLSNYYINWVRQAPGKGLEWVAIIFCAGNAYNASWAKGRFTISRDDSKNTLYLQMNSLRAEDTAVYYCARGWQALVNWGQGTLVTVSSASTKGPSVFPLAPSSKSTSGGTAALGCLVKDYFPEPVTVSWNSGALTSGVHTFPAVLQSSGLYSLSSVVTVPSSSLGTQTYICNVNHKPSNTKVDKRVEPKSCDK

SEQ ID NO: 120 - protein, 254 aa, Artificial Sequence
  Synthetic
GGGSGGGEVQLVESGGGLVQPGGSLRLSCAASGFSLSNYYINWVRQAPGKGLEWVAIIFCAGNAYNASWAKGRFTISRDDSKNTLYLQMNSLRAEDTAVYYCARGWQALVNWGQGTLVTVSSGGGGSGGGGSGGGGSDIQMTQSPSSLSASVGDRVTITCQASQSISSSYLSWYQQKPGKAPKLLIYAVSYLASGVPSRFSGSGSGTDFTLTISSLQPEDFATYYCQSGYYSAGDLTFGQGTKVEIKRHHHHHH

SEQ ID NO: 121 - protein, 241 aa, Artificial Sequence
  Synthetic
DIQMTQSPSSLSASVGDRVTITCQASQSISSSYLSWYQQKPGKAPKLLIYAVSYLASGVPSRFSGSGSGTDFTLTISSLQPEDFATYYCQSGYYSAGDLTFGQGTKVEIKRGGGGSGGGGSGGGGSEVQLVESGGGLVQPGGSLRLSCAASGFSLSNYYINWVRQAPGKGLEWVAIIFCAGNAYNASWAKGRFTISRDDSKNTLYLQMNSLRAEDTAVYYCARGWQALVNWGQGTLVTVSS

SEQ ID NO: 122 - protein, 230 aa, Artificial Sequence
  Synthetic
RIQMTQSPSSLSASVGDRVTITCQASQSISSSYLSWYQDKPGKAPKLLIYAVSYLASGVPSRFSGSGSGTDFTLTISSLQPEDFATYYCQSGYYSAGDLTFGQGTKVEIKRTVAAPSVFIFPPSDEQLKSGTASVVCYLNNFYPREAKVQWKVDNALQSGNSQESVTEQDSKDSTYSLWSTLTLSKADYEKHKLYACEVTHQGLSSPVTKSFNRGECGGGSYPYDVPDYA

SEQ ID NO: 123 - protein, 445 aa, Artificial Sequence
  Synthetic
EVQLVESGGGLVQPGGSLRLSCAASGFSLSNYYINWVRKAPGKGLEWVAIIFCAGNAYNASWAKGEFTISRDDSKNTLYLQMNSLRAEDTAVYYCARGWQALVNWGQGTLVTVSSASTKGPSVFPLAPSSKSTSGGTAALGCLVKDYFPEPVTVSWNSGALTSGVATGPAVLQSSGLYSLSSVVTVPSSSLGTQTYICNVNHKPSNTKVDKKVEPKSCDKTHTCPPCPAPELLGGPSVFLFPPKPKDTLMISRTPEVTCVVVDVSHEDPEVKFNWYVDGVEVHNAKTKPREEQYNSTYRVVSVLTVLHQDWLNGKEYKCKVSNKALPAPIEKTISKAKGQPREPQVYTLPPSRKELTKNQVSLTCLVKGFYPSDIAVEWESNGQPENNYKTTPPVLKSDGSFFLYSKLTVDKSRWQQGNVFSCSVMHEALHNHYTQKSLSLSPGK

SEQ ID NO: 124 - protein, 119 aa, Artificial Sequence
  Synthetic
QVQLVQSGAEVKKPGASVKVSCKASGYTFTRYTMHWVRQAPGQGLEWMGYINPSRGYTSYAQKFQGRVTMTTDKSTSTVYMELSSLRSEDTAVYYCARYYDDHYCLDYWGQGTTVTVSS

SEQ ID NO: 125 - protein, 5 aa, Artificial Sequence
  Synthetic
RYTMH

SEQ ID NO: 126 - protein, 17 aa, Artificial Sequence
  Synthetic
YINPSRGYTSYAQKFQG

SEQ ID NO: 127 - protein, 10 aa, Artificial Sequence
  Synthetic
YYDDHYCLDY

SEQ ID NO: 128 - protein, 107 aa, Artificial Sequence
  Synthetic
DIQMTQSPSSLSASVGDRVTITCRASSSVSYMNWYQQKPGKAPKLLIYDTSKVASGVPSRFSGSGSGTDYTLTISSLQPEDFATYYCQQWSSNPLTFGGGTKVEIKR

SEQ ID NO: 129 - protein, 10 aa, Artificial Sequence
  Synthetic
RASSSVSYMN

SEQ ID NO: 130 - protein, 7 aa, Artificial Sequence
  Synthetic
DTSKVAS

SEQ ID NO: 131 - protein, 9 aa, Artificial Sequence
  Synthetic
QQWSSNPLT

SEQ ID NO: 132 - DNA, 774 bp, Artificial Sequence
  Synthetic
ggtggcggctcaggtggaggccaggtgcagctggtgcagagcggcgcggaagtgaaaaaaccgggcgcgagcgtgaaagtgagctgcaaagcgagcggctatacctttacccgctataccatgcattgggtgcgccaggcgccgggccagggcctggaatggatgggctatattaacccgagccgcggctataccagctatgcgcagaaatttcagggccgcgtgaccatgaccaccgataaaagcaccagcaccgtgtatatggaactgagcagcctgcgcagcgaagataccgcggtgtattattgcgcgcgctattatgatgatcattattgcctggattattggggccagggcaccaccgtgaccgtgagcagcgtggagggcggcagcggcggcagcggcggcagcggcggcagcggcggcgtggacgatattcagatgacccagagcccgagcagcctgagcgcgagcgtgggcgatcgcgtgaccattacctgccgcgcgagcagcagcgtgagctatatgaactggtatcagcagaaaccgggcaaagcgccgaaactgctgatttatgataccagcaaagtggcgagcggcgtgccgagccgctttagcggcagcggcagcggcaccgattataccctgaccattagcagcctgcagccggaagattttgcgacctattattgccagcagtggagcagcaacccgctgacctttggcggcggcaccaaagtggaaattaaacgccaccaccaccaccaccactga

SEQ ID NO: 133 - protein, 257 aa, Artificial Sequence
  Synthetic
GGGSGGGQVQLVQSGAEVKKPGASVKVSCKASGYTFTRYTMHWVRQAPGQGLEWMGYINPSRGYTSYAQKFQGRVTMTTDKSTSTVYMELSSLRSEDTAVYYCARYYDDHYCLDYWGQGTTVTVSSVEGGSGGSGGSGGSGGVDDIQMTQSPSSLSASVGDRVTITCRASSSVSYMNWYQQKPGKAPKLLIYDTSKVASGVPSRFSGSGSGTDYTLTISSLQPEDFATYYCQQWSSNPLTFGGGTKVEIKRHHHHHH

SEQ ID NO: 134 - DNA, 642 bp, Artificial Sequence
  Synthetic
gatattcagatgacccagagcccgagcagcctgagcgcgagcgtgggcgatcgcgtgaccattacctgccgcgcgagcagcagcgtgagctatatgaactggtatcagcagaaaccgggcaaagcgccgaaactgctgatttatgataccagcaaagtggcgagcggcgtgccgagccgctttagcggcagcggcagcggcaccgattataccctgaccattagcagcctgcagccggaagattttgcgacctattattgccagcagtggagcagcaacccgctgacctttggcggcggcaccaaagtggaaattaaacgcactgtggctgcaccatctgtcttcatcttcccgccatctgatgagcagttgaaatctggaactgcctctgttgtgtgcctgctgaataacttctatcccagagaggccaaagtacagtggaaggtggataacgccctccaatcgggtaactcccaggagagtgtcacagagcaggacagcaaggacagcacctacagcctcagcagcaccctgacgctgagcaaagcagactacgagaaacacaaactctacgcctgcgaagtcacccatcagggcctgagctcgcccgtcacaaagagcttcaacaggggagagtgctga

SEQ ID NO: 135 - protein, 213 aa, Artificial Sequence
  Synthetic
DIQMTQSPSSLSASVGDRVTITCRASSSVSYMNWYQQKPGKAPKLLIYDTSKVASGVPSRFSGSGSGTDYTLTISSLQPEDFATYYCQQWSSNPLTFGGGTKVEIKRTVAAPSVFIFPPSDEQLKSGTASVVCLLNNFYPREAKVQWKVDNALQSGNSQESVTEQDSKDSTYSLSSTLTLSKADYEKHKLYACEVTHQGLSSPVTKSFNRGEC

SEQ ID NO: 136 - DNA, 651 bp, Artificial Sequence
  Synthetic
caggtgcagctggtgcagagcggcgcggaagtgaaaaaaccgggcgcgagcgtgaaagtgagctgcaaagcgagcggctatacctttacccgctataccatgcattgggtgcgccaggcgccgggccagggcctggaatggatgggctatattaacccgagccgcggctataccagctatgcgcagaaatttcagggccgcgtgaccatgaccaccgataaaagcaccagcaccgtgtatatggaactgagcagcctgcgcagcgaagataccgcggtgtattattgcgcgcgctattatgatgatcattattgcctggattattggggccagggcaccaccgtgaccgtgagcagcgcctccaccaaaggtccatcggtcttccccctggcgccctgctccaggagcacctccgagagcacagcggccctgggctgcctggtcaaggactacttccccgaaccggtgacggtgtcgtggaactcaggcgctctgaccagcggcgtgcacaccttcccagctgtcctacagtcctcaggactctactccctcagcagcgtggtgaccgtgccctccagcaacttcggcacccagacctacacctgcaacgtagatcacaagcccagtaacaccaaggtggacaagacagtt

SEQ ID NO: 137 - protein, 217 aa, Artificial Sequence
  Synthetic
QVQLVQSGAEVKKPGASVKVSCKASGYTFTRYTMHWVRQAPGQGLEWMGYINPSRGYTSYAQKFQGRVTMTTDKSTSTVYMELSSLRSEDTAVYYCARYYDDHYCLDYWGQGTTVTVSSASTKGPSVFPLAPCSRSTSESTAALGCLVKDYFPEPVTVSWNSGALTSGVHTFPAVLQSSGLYSLSSVVTVPSSNFGTQTYTCNVDHKPSNTKVDKTV

SEQ ID NO: 138 - DNA, 765 bp, Artificial Sequence
  Synthetic
ggcggtggatcacaggtgcagctggtgcagagcggcgcggaagtgaaaaaaccgggcgcgagcgtgaaagtgagctgcaaagcgagcggctatacctttacccgctataccatgcattgggtgcgccaggcgccgggccagggcctggaatggatgggctatattaacccgagccgcggctataccagctatgcgcagaaatttcagggccgcgtgaccatgaccaccgataaaagcaccagcaccgtgtatatggaactgagcagcctgcgcagcgaagataccgcggtgtattattgcgcgcgctattatgatgatcattattgcctggattattggggccagggcaccaccgtgaccgtgagcagcgtggagggcggcagcggcggcagcggcggcagcggcggcagcggcggcgtggacgatattcagatgacccagagcccgagcagcctgagcgcgagcgtgggcgatcgcgtgaccattacctgccgcgcgagcagcagcgtgagctatatgaactggtatcagcagaaaccgggcaaagcgccgaaactgctgatttatgataccagcaaagtggcgagcggcgtgccgagccgctttagcggcagcggcagcggcaccgattataccctgaccattagcagcctgcagccggaagattttgcgacctattattgccagcagtggagcagcaacccgctgacctttggcggcggcaccaaagtggaaattaaacgccaccaccaccaccaccactga

SEQ ID NO: 139 - protein, 254 aa, Artificial Sequence
  Synthetic
GGGSQVQLVQSGAEVKKPGASVKVSCKASGYTFTRYTMHWVRQAPGQGLEWMGYINPSRGYTSYAQKFQGRVTMTTDKSTSTVYMELSSLRSEDTAVYYCARYYDDHYCLDYWGQGTTVTVSSVEGGSGGSGGSGGSGGVDDIQMTQSPSSLSASVGDRVTITCRASSSVSYMNWYQQKPGKAPKLLIYDTSKVASGVPSRFSGSGSGTDYTLTISSLQPEDFATYYCQQWSSNPLTFGGGTKVEIKRHHHHHH

SEQ ID NO: 140 - DNA, 672 bp, Artificial Sequence
  Synthetic
gatattcagatgacccagagcccgagcagcctgagcgcgagcgtgggcgatcgcgtgaccattacctgccgcgcgagcagcagcgtgagctatatgaactggtatcagcgtaaaccgggcaaagcgccgaaactgctgatttatgataccagcaaagtggcgagcggcgtgccgagccgctttagcggcagcggcagcggcaccgattataccctgaccattagcagcctgcagccggaagattttgcgacctattattgccagcagtggagcagcaacccgctgacctttggcggcggcaccaaagtggaaattaaacgcaccgtggcagcacctagcgtgttcatctttcccccttccgacgagcagctgaagtccggcacagcctctgtggtgtgcctgctgaacaatttctatccacgcgaggccaaggtgcagtggaaggtggataacgccctgcagtctggcaatagccaggagtccgtgaccgagcaggactctaaggatagcacatactccctgtcctctaccctgacactgagcaaggccgattacgagaagcacaagctgtatgcatgcgaggtgacccaccagggcctgagctccccagtgacaaagtcttttaaccggggcgagtgtggcggcggctcccaccaccaccaccaccactga

SEQ ID NO: 141 - protein, 223 aa, Artificial Sequence
  Synthetic
DIQMTQSPSSLSASVGDRVTITCRASSSVSYMNWYQRKPGKAPKLLIYDTSKVASGVPSRFSGSGSGTDYTLTISSLQPEDFATYYCQQWSSNPLTFGGGTKVEIKRTVAAPSVFIFPPSDEQLKSGTASVVCLLNNFYPREAKVQWKVDNALQSGNSQESVTEQDSKDSTYSLSSTLTLSKADYEKHKLYACEVTHQGLSSPVTKSFNRGECGGGSHHHHHH

SEQ ID NO: 142 - DNA, 1350 bp, Artificial Sequence
  Synthetic
caggtgcagctggtgcagagcggcgcggaagtgaaaaaaccgggcgcgagcgtgaaagtgagctgcaaagcgagcggctatacctttacccgctataccatgcattgggtgcgctatgcgccgggccagggcctggaatggatgggctatattaacccgagccgcggctataccagctatgcgcagaaatttcagggccgcgtgaccatgaccaccgataaaagcaccagcaccgtgtatatggaactgagcagcctgcgcagcgaagataccgcggtgtattattgcgcgcgctattatgatgatcattattgcctggattattggggccagggcaccaccgtgaccgtgagcagcgcctctacaaagggacctagcgtgttcccactggcaccctcctctaagtccacctctggaggaacagccgccctgggatgcctggtgaaggattacttcccagagcccgtgaccgtgtcctggaactctggcgccctgaccagcggagtgcacacatttcctgccgtgctgcagagctccggcctgtactccctgtctagcgtggtgacagtgccatcctctagcctgggcacccagacatatatctgcaacgtgaatcacaagccaagcaataccaaggtcgacaagaaggtggagcccaagtcctgtgataagacccacacatgccccccttgtcctgcaccagagctgctgggaggaccaagcgtgttcctgtttccacccaagcctaaggacaccctgatgatctctcggaccccagaggtgacatgcgtggtggtggacgtgagccacgaggatcccgaggtgaagtttaactggtacgtggatggcgtggaggtgcacaatgccaagaccaagcccagggaggagcagtacaattccacctatcgcgtggtgtctgtgctgacagtgctgcaccaggactggctgaacggcaaggagtataagtgcaaggtgtccaataaggccctgcccgcccctatcgagaagacaatctctaaggcaaagggacagcctcgggagccacaggtgtacaccctgcctccatccagagatgagctgaccaagaaccaggtgtctctgacatgtctggtgaagggcttctatccctctgacatcgccgtggagtgggagagcaatggccagcctgagaacaattacgataccacaccccctgtgctggacagcgatggctccttctttctgtatagcgacctgacagtggataagtccagatggcagcagggcaacgtgtttagctgttccgtgatgcacgaggccctgcacaatcactacacccagaagtctctgagcctgtcccccggcaagtaa

SEQ ID NO: 143 - protein, 449 aa, Artificial Sequence
  Synthetic
QVQLVQSGAEVKKPGASVKVSCKASGYTFTRYTMHWVRYAPGQGLEWMGYINPSRGYTSYAQKFQGRVTMTTDKSTSTVYMELSSLRSEDTAVYYCARYYDDHYCLDYWGQGTTVTVSSASTKGPSVFPLAPSSKSTSGGTAALGCLVKDYFPEPVTVSWNSGALTSGVHTFPAVLQSSGLYSLSSVVTVPSSSLGTQTYICNVNHKPSNTKVDKKVEPKSCDKTHTCPPCPAPELLGGPSVFLFPPKPKDTLMISRTPEVTCVVVDVSHEDPEVKFNWYVDGVEVHNAKTKPREEQYNSTYRVVSVLTVLHQDWLNGKEYKCKVSNKALPAPIEKTISKAKGQPREPQVYTLPPSRDELTKNQVSLTCLVKGFYPSDIAVEWESNGQPENNYDTTPPVLDSDGSFFLYSDLTVDKSRWQQGNVFSCSVMHEALHNHYTQKSLSLSPGK